European Patent Specification EP 3 673 062 B1, published September 6, 2023. Title: Multi-copy gene protein expression system. Applicant: Sandoz AG. The sequence listing filed with the application follows.

SEQUENCE LISTING (10 sequences)

SEQ ID NO: 1 - DNA, 4355 bp, Artificial Sequence
  synthetic vector sequence
cccgtagaaaagatcaaaggatcttcttgagatcctttttttctgcgcgtaatctgctgcttgcaaacaaaaaaaccaccgctaccagcggtggtttgtttgccggatcaagagctaccaactctttttccgaaggtaactggcttcagcagagcgcagataccaaatactgttcttctagtgtagccgtagttaggccaccacttcaagaactctgtagcaccgcctacatacctcgctctgctaatcctgttaccagtggctgctgccagtggcgataagtcgtgtcttaccgggttggactcaagacgatagttaccggataaggcgcagcggtcgggctgaacggggggttcgtgcacacagcccagcttggagcgaacgacctacaccgaactgagatacctacagcgtgagctatgagaaagcgccacgcttcccgaagggagaaaggcggacaggtatccggtaagcggcagggtcggaacaggagagcgcacgagggagcttccagggggaaacgcctggtatctttatagtcctgtcgggtttcgccacctctgacttgagcgtcgatttttgtgatgctcgtcaggggggcggagcctatggaaaaacgccagcaacgcggcctttttacggttcctggccttttgctggccttttgctcacatgttctttcctgcggtacccagatccaattcccgctttgactgcctgaaatctccatcgcctacaatgatgacatttggatttggttgactcatgttggtattgtgaaatagacgcagatcgggaacactgaaaaatacacagttattattcatttaaatcacggtcttggagtcatcaggctctgactgggcagctgctgcaactggaacttcccaagcctcccaccaaacagcaggtgtagccgaaagtattcacgtgtcccagaatgaggcccacagtacatctgtcaccgtttctcaacccccttcaacggtttctttgcaaattggagaagcaaataccctgaaatggtcagctttctttggagtagtagttccgctgctcaacgtactcttcgtttaaaagccctcctaggacaaaatggccaagctgggaaacgggatttggtggaactttattattctttctacgatccaagcattatgttgtggaacaaagcgaatactcttattagctggtaattgagcgagttgaaaaaatcaagtctattggagggtatggtcagagtactgatagagatccctgttaagataatcgatctttttcaaatatccaatttcattccatcttgccatcgggtcttggcttcttacatcaataattaaaactacttactctattagtgccaaaaatggtaaaccgtattcaaattgctgcaagcatatgcttaaaaggatcgcgttgcgagcttcttttgagattcgcaagcttgattttatgctcttgtgggaagaaaagcaacccactgaattccagatttgttgtgttttcatgcatggacgacatactttgagtaataccgttactgagattttaccgaattcgcattgcgttgaggcgtgaagtttcttaatgctgtgccatatggttaagttgcgtttcaagatggtccacaagtatttttgtatttaagcagtgtcaattcaagcctaactgctcataaaaactacacggtttgctgatatcaaaaacgatgtttgagaagagtaaatttgtggtttcgtttctgcttttactccagctattttgtgtccttggtgtacatggagaaattgtcatgacccaaagtccatcaactctttctgcctcagttggtgatagagttatcattacttgtcagagttctcaatctgtgttcaacaattacttgagctggtaccaacaaaaacctggtagagcccccaaactgttaatctacgatgcatccaaactggctagcggagtaccttctaggtttagcggttccggatcaggtgcagaatttacactgacaatatcctctttgcaaccagacgactttgccacatactattgccaaggttcggattatagcggtggttgggactccgcgtttggtcaaggtaccaagttgactgttctcggtggaggtggaggttctggtggtggaggatcaggtggtggcggatctggcggtggagggtccgaggtgcagttggtagagtcgggcggtggatcagtccagcctggtggatccttgagactttcctgtaccgcttctggtatcgacttatccagttatcccatgtcgtgggttagacaagctccgggaaagggtttggaatgggttggtatcatcagcactagaggaaatacttactacgctacttgggctaagggacgttttacaattagtagagatacgtctaaaaacactgtgtatttgcagatgaattcactaagagccgaggacactgcaacttactactgtgcacgtggtctttacggtaataactattatggagctttcaatttgtggggacaaggcacaactgtaacggtgtcctcataataagcggccgcagcgaatttcttatgatttatgatttttattattaaataagttataaaaaaaataagtgtatacaaattttaaagtgactcttaggttttaaaacgaaaattcttattcttgagtaactctttcctgtaggtcaggttgctttctcaggtatagcatgaggtcgctcttattgaccacacctctaccggcatgccgagcaaatgcctgcaaatcgctccccatttcacccaattgtagatatgctaactccagcaatgagttgatgaatctcggtgtgtattttatgtcctcagaggacaaggatccttcagtaatgtcttgtttcttttgttgcagtggtgagccattttgacttcgtgaaagtttctttagaatagttgtttccagaggccaaacattccacccgtagtaaagtgcaagcgtaggaagaccaagactggcataaatcaggtataagtgtcgagcactggcaggtgatcttctgaaagtttctactagcagataagatccagtagtcatgcatatggcaacaatgtaccgtgtggatctaagaacgcgtcctactaaccttcgcattcgttggtccagtttgttgttatcgatcaacgtgacaaggttgtcgattccgcgtaagcatgcatacccaaggacgcctgttgcaattccaagtgagccagttccaacaatctttgtaatattagagcacttcattgtgttgcgcttgaaagtaaaatgcgaacaaattaagagataatctcgaaaccgcgacttcaaacgccaatatgatgtgcggcacacaataagcgttcatatccgctgggtgactttctcgctttaaaaaattatccgaaaaaattttctagagtgttgacactttatacttccggctcgtataatacgacaaggtgtaaggaggactaaaccatggctaaactcacctctgctgttccagtcctgactgctcgtgatgttgctggtgctgttgagttctggactgatagactcggtttctcccgtgacttcgtagaggacgactttgccggtgttgtacgtgacgacgttaccctgttcatctccgcagttcaggaccaggttgtgccagacaacactctggcatgggtatgggttcgtggtctggacgaactgtacgctgagtggtctgaggtcgtgtctaccaacttccgtgatgcatctggtccagctatgaccgagatcggtgaacagccctggggtcgtgagtttgcactgcgtgatccagctggtaactgcgtgcatttcgtcgcagaagagcaggactaacctctaggacaccttacgattatttagagagtatttattagttttattgtatgtatacggatgttttattatctatttatgcccttatattctgtaactatccaaaagtcctatcttatcaagccagcaatctatgtccgcgaacgtcaactaaaaataagctttttatgctcttctctctttttttcccttcggtataattataccttgcatccacagattctcctgccaaattttgcataatcctttacaacatggctatatgggagcacttagcgccctccaaaacccatattgcctacgcatgtataggtgttttttccacaatattttctctgtgctctctttttattaaagagaagctctatatcggagaagcttctgtggccgttatattcggccttatcgtgggaccacattgcctgaattggtttgccccggaagattggggaaacttggatctgattaccttagctgcaggtaccactgagcgtcagac

SEQ ID NO: 2 - DNA, 5904 bp, Artificial Sequence
  synthetic vector sequence
cccgtagaaaagatcaaaggatcttcttgagatcctttttttctgcgcgtaatctgctgcttgcaaacaaaaaaaccaccgctaccagcggtggtttgtttgccggatcaagagctaccaactctttttccgaaggtaactggcttcagcagagcgcagataccaaatactgttcttctagtgtagccgtagttaggccaccacttcaagaactctgtagcaccgcctacatacctcgctctgctaatcctgttaccagtggctgctgccagtggcgataagtcgtgtcttaccgggttggactcaagacgatagttaccggataaggcgcagcggtcgggctgaacggggggttcgtgcacacagcccagcttggagcgaacgacctacaccgaactgagatacctacagcgtgagctatgagaaagcgccacgcttcccgaagggagaaaggcggacaggtatccggtaagcggcagggtcggaacaggagagcgcacgagggagcttccagggggaaacgcctggtatctttatagtcctgtcgggtttcgccacctctgacttgagcgtcgatttttgtgatgctcgtcaggggggcggagcctatggaaaaacgccagcaacgcggcctttttacggttcctggccttttgctggccttttgctcacatcgcgatagaatagccgtatgggctttttgtagaaatgtcttggtgtcctcgtccaatcaggtagccatctctgaaatatctggctccgttgcaactccgaacgacctgctggcaacgtaaaattctccggggtaaaacttaaatgtggagtaatggaaccagaaacgtctcttcccttctctctccttccaccgcccgttaccgtcactaggaaattttactctgctggagagcttcttctacggcccccttgcagcaatgctcttcccagcattacgttgcgggtaaaacggaggtcgtgtacccgacctagcagcccagggatggaaaagtcccggccgtcgctggcaataatagcgggcggacgcatgtcatgagattattggaaaccaccagaatcgaatataaaaggcgaacacctttcccaattttggtttctcctgacccaaagactttaaatttaatttatttgtccctatttcaatcaattgaacaactatcaaaacacactcgagcaaaacgatgcgtttcccatcgattttcacagctgttctgtttgcagcttcatctgctttagctgcacctgttaacacaactacagaggacgaaacggcccagatcccagctgaggcagtcattggttattccgatttggaaggtgatttcgatgtcgctgtgttaccattcagtaattccacaaataacggtttgctgttcattaacaccactatagcaagcatcgctgcaaaagaggaaggtgtttccctagaaaagagggagattgttatgacgcagtcccccagtactttgtctgcttccgttggagatagagtaatcataacttgtcaatcctctcaatctgtctttaacaattacctttcttggtaccaacagaaaccaggcagggctccaaagttgctaatctatgatgcatctaaactggcctccggtgttccatcacgtttttcaggttcaggatccggtgctgagttcactttaacgatttcctcgttgcaaccggatgactttgccacatattactgtcaaggttctgactactcaggtggttgggactctgctttcggtcaaggtaccaaactgactgtattgggaggaggtggaggtagcggcggtggaggttcaggaggtggtggatccggagggggtggaagtgaagttcaattggtggaaagcggtggtggttccgttcagcctggaggtagcttgcgtctgtcgtgcactgcaagtggtattgacttaagctcatatcctatgtcttgggtcagacaagcacctggtaagggtttggagtgggtcggcatcattagcactagaggtaacacatactatgctacatgggcaaagggaagattcacaatctcacgtgatacatctaaaaatacagtttatcttcagatgaatagtctcagagctgaagatacagctacctactactgtgccagaggattatacggtaataactattatggtgcattcaatctatggggccaaggtactactgtgaccgtgtcctcgtaatagaggccttgttctttcctgcggtacccagatccaattcccgctttgactgcctgaaatctccatcgcctacaatgatgacatttggatttggttgactcatgttggtattgtgaaatagacgcagatcgggaacactgaaaaatacacagttattattcatttaaatcacggtcttggagtcatcaggctctgactgggcagctgctgcaactggaacttcccaagcctcccaccaaacagcaggtgtagccgaaagtattcacgtgtcccagaatgaggcccacagtacatctgtcaccgtttctcaacccccttcaacggtttctttgcaaattggagaagcaaataccctgaaatggtcagctttctttggagtagtagttccgctgctcaacgtactcttcgtttaaaagccctcctaggacaaaatggccaagctgggaaacgggatttggtggaactttattattctttctacgatccaagcattatgttgtggaacaaagcgaatactcttattagctggtaattgagcgagttgaaaaaatcaagtctattggagggtatggtcagagtactgatagagatccctgttaagataatcgatctttttcaaatatccaatttcattccatcttgccatcgggtcttggcttcttacatcaataattaaaactacttactctattagtgccaaaaatggtaaaccgtattcaaattgctgcaagcatatgcttaaaaggatcgcgttgcgagcttcttttgagattcgcaagcttgattttatgctcttgtgggaagaaaagcaacccactgaattccagatttgttgtgttttcatgcatggacgacatactttgagtaataccgttactgagattttaccgaattcgcattgcgttgaggcgtgaagtttcttaatgctgtgccatatggttaagttgcgtttcaagatggtccacaagtatttttgtatttaagcagtgtcaattcaagcctaactgctcataaaaactacacggtttgctgatatcaaaaacgatgtttgagaagagtaaatttgtggtttcgtttctgcttttactccagctattttgtgtccttggtgtacatggagaaattgtcatgacccaaagtccatcaactctttctgcctcagttggtgatagagttatcattacttgtcagagttctcaatctgtgttcaacaattacttgagctggtaccaacaaaaacctggtagagcccccaaactgttaatctacgatgcatccaaactggctagcggagtaccttctaggtttagcggttccggatcaggtgcagaatttacactgacaatatcctctttgcaaccagacgactttgccacatactattgccaaggttcggattatagcggtggttgggactccgcgtttggtcaaggtaccaagttgactgttctcggtggaggtggaggttctggtggtggaggatcaggtggtggcggatctggcggtggagggtccgaggtgcagttggtagagtcgggcggtggatcagtccagcctggtggatccttgagactttcctgtaccgcttctggtatcgacttatccagttatcccatgtcgtgggttagacaagctccgggaaagggtttggaatgggttggtatcatcagcactagaggaaatacttactacgctacttgggctaagggacgttttacaattagtagagatacgtctaaaaacactgtgtatttgcagatgaattcactaagagccgaggacactgcaacttactactgtgcacgtggtctttacggtaataactattatggagctttcaatttgtggggacaaggcacaactgtaacggtgtcctcataataagcggccgcagcgaatttcttatgatttatgatttttattattaaataagttataaaaaaaataagtgtatacaaattttaaagtgactcttaggttttaaaacgaaaattcttattcttgagtaactctttcctgtaggtcaggttgctttctcaggtatagcatgaggtcgctcttattgaccacacctctaccggcatgccgagcaaatgcctgcaaatcgctccccatttcacccaattgtagatatgctaactccagcaatgagttgatgaatctcggtgtgtattttatgtcctcagaggacaaggatccttcagtaatgtcttgtttcttttgttgcagtggtgagccattttgacttcgtgaaagtttctttagaatagttgtttccagaggccaaacattccacccgtagtaaagtgcaagcgtaggaagaccaagactggcataaatcaggtataagtgtcgagcactggcaggtgatcttctgaaagtttctactagcagataagatccagtagtcatgcatatggcaacaatgtaccgtgtggatctaagaacgcgtcctactaaccttcgcattcgttggtccagtttgttgttatcgatcaacgtgacaaggttgtcgattccgcgtaagcatgcatacccaaggacgcctgttgcaattccaagtgagccagttccaacaatctttgtaatattagagcacttcattgtgttgcgcttgaaagtaaaatgcgaacaaattaagagataatctcgaaaccgcgacttcaaacgccaatatgatgtgcggcacacaataagcgttcatatccgctgggtgactttctcgctttaaaaaattatccgaaaaaattttctagagtgttgacactttatacttccggctcgtataatacgacaaggtgtaaggaggactaaaccatggctaaactcacctctgctgttccagtcctgactgctcgtgatgttgctggtgctgttgagttctggactgatagactcggtttctcccgtgacttcgtagaggacgactttgccggtgttgtacgtgacgacgttaccctgttcatctccgcagttcaggaccaggttgtgccagacaacactctggcatgggtatgggttcgtggtctggacgaactgtacgctgagtggtctgaggtcgtgtctaccaacttccgtgatgcatctggtccagctatgaccgagatcggtgaacagccctggggtcgtgagtttgcactgcgtgatccagctggtaactgcgtgcatttcgtcgcagaagagcaggactaacctctaggacaccttacgattatttagagagtatttattagttttattgtatgtatacggatgttttattatctatttatgcccttatattctgtaactatccaaaagtcctatcttatcaagccagcaatctatgtccgcgaacgtcaactaaaaataagctttttatgctcttctctctttttttcccttcggtataattataccttgcatccacagattctcctgccaaattttgcataatcctttacaacatggctatatgggagcacttagcgccctccaaaacccatattgcctacgcatgtataggtgttttttccacaatattttctctgtgctctctttttattaaagagaagctctatatcggagaagcttctgtggccgttatattcggccttatcgtgggaccacattgcctgaattggtttgccccggaagattggggaaacttggatctgattaccttagctgcaggtaccactgagcgtcagac

SEQ ID NO: 3 - DNA, 7866 bp, Artificial Sequence
  synthetic vector sequence
cgatttattatgttacaatatggaagggaactttacacttctcctatgcacatatattaattaaagtccaatgctagtagagaaggggggtaacacccctccgcgctcttttccgatttttttctaaaccgtggaatatttcgcatatccttttgttgtttccgggtgtacaatatggacttcctcttttctggcaaccaaacccatacatcgggattcctataataccttcgttggtctccctaacatgtaggtggcggaggggagatatacaatagaacagataccagacaagacataatgggctaaacaagactacaccaattacactgcctcattgatggtggtacataacgaactaatactgtagccctagacttgatagccatcatcatatcgaagtttcactaccctttttccatttgccatctattgaagtaataataggcgcatgcaacttcttttctttttttttcttttctctctcccccgttgttgtctcaccatatccgcaatgacaaaaaaatgatggaagacactaaaggaaaaaattaacgacaaagacagcaccaacagatgtcgttgttccagagctgatgaggggtatctcgaagcacacgaaactttttccttccttcattcacgcacactactctctaatgagcaacggtatacggccttccttccagttacttgaatttgaaataaaaaaaagtttgctgtcttgctatcaagtataaatagacctgcaattattaatcttttgtttcctcgtcattgttctcgttccctttcttccttgtttctttttctgcacaatatttcaagctataccaagcatacaatcaactatctcatatacagtcgaccaaaacgatgaagtgggtcactttcatctcgctgctatttttgttctccagcgcctatagcgagattgtgatgactcaatccccttccactctaagcgcttctgtcggtgaccgtgttatcattacctgtcaatcctctcaatcggttttcaacaattacttatcctggtatcaacagaagccaggtcgtgcacctaaacttctgatttacgatgcttcaaaattggctagtggtgtcccaagcagattttcgggatctggttccggtgccgagtttacactcacgatctcctcacttcaacccgatgatttcgcaacatactattgtcaaggtagcgactatagtggaggttgggactctgcctttggacaaggtactaagctaacagttttgggtggaggcggaggttcgggtggtggtggatcaggaggaggtggtagtggcggaggaggctcagaagtgcaactggttgaaagtggtggaggttccgttcagccagggggttccttgagattgtcttgcactgcttctggtatcgacctgtcatcatacccaatgagctgggtaagacaggctcctggtaaaggtttggaatgggttggaattatctctactcgtggtaatacatattacgcaacatgggctaagggtagattcacaatatccagggatacttccaaaaacacagtatacttacaaatgaattctttgagagccgaggataccgctacctattactgtgcaaggggtctgtatggtaacaattactatggagcattcaatttgtggggtcagggcacgactgtgactgtcagctcataatagagatctccttttcctttgtccatatcatgtaattagttatgtcacgcttacattcacgccctccccccacatccgctctaaccgaaaaggaaggagttagacaacctgaagtctaggtccctatttatttttttatagttatgttagtattaagaacgttatttatatttcaaatttttcttttttttctgtacagacgcgtgtacgcatgtaacattatactgaaaaccttgcttgagaaggttttgggacgctcgaaggctttaatttgcaagctgccgtatgggctttttgtagaaatgtcttggtgtcctcgtccaatcaggtagccatctctgaaatatctggctccgttgcaactccgaacgacctgctggcaacgtaaaattctccggggtaaaacttaaatgtggagtaatggaaccagaaacgtctcttcccttctctctccttccaccgcccgttaccgtcactaggaaattttactctgctggagagcttcttctacggcccccttgcagcaatgctcttcccagcattacgttgcgggtaaaacggaggtcgtgtacccgacctagcagcccagggatggaaaagtcccggccgtcgctggcaataatagcgggcggacgcatgtcatgagattattggaaaccaccagaatcgaatataaaaggcgaacacctttcccaattttggtttctcctgacccaaagactttaaatttaatttatttgtccctatttcaatcaattgaacaactatcaaaacacactcgagcaaaacgatgcgtttcccatcgattttcacagctgttctgtttgcagcttcatctgctttagctgcacctgttaacacaactacagaggacgaaacggcccagatcccagctgaggcagtcattggttattccgatttggaaggtgatttcgatgtcgctgtgttaccattcagtaattccacaaataacggtttgctgttcattaacaccactatagcaagcatcgctgcaaaagaggaaggtgtttccctagaaaagagggagattgttatgacgcagtcccccagtactttgtctgcttccgttggagatagagtaatcataacttgtcaatcctctcaatctgtctttaacaattacctttcttggtaccaacagaaaccaggcagggctccaaagttgctaatctatgatgcatctaaactggcctccggtgttccatcacgtttttcaggttcaggatccggtgctgagttcactttaacgatttcctcgttgcaaccggatgactttgccacatattactgtcaaggttctgactactcaggtggttgggactctgctttcggtcaaggtaccaaactgactgtattgggaggaggtggaggtagcggcggtggaggttcaggaggtggtggatccggagggggtggaagtgaagttcaattggtggaaagcggtggtggttccgttcagcctggaggtagcttgcgtctgtcgtgcactgcaagtggtattgacttaagctcatatcctatgtcttgggtcagacaagcacctggtaagggtttggagtgggtcggcatcattagcactagaggtaacacatactatgctacatgggcaaagggaagattcacaatctcacgtgatacatctaaaaatacagtttatcttcagatgaatagtctcagagctgaagatacagctacctactactgtgccagaggattatacggtaataactattatggtgcattcaatctatggggccaaggtactactgtgaccgtgtcctcgtaatagaggccttgttctttcctgcggtacccagatccaattcccgctttgactgcctgaaatctccatcgcctacaatgatgacatttggatttggttgactcatgttggtattgtgaaatagacgcagatcgggaacactgaaaaatacacagttattattcatttaaatcacggtcttggagtcatcaggctctgactgggcagctgctgcaactggaacttcccaagcctcccaccaaacagcaggtgtagccgaaagtattcacgtgtcccagaatgaggcccacagtacatctgtcaccgtttctcaacccccttcaacggtttctttgcaaattggagaagcaaataccctgaaatggtcagctttctttggagtagtagttccgctgctcaacgtactcttcgtttaaaagccctcctaggacaaaatggccaagctgggaaacgggatttggtggaactttattattctttctacgatccaagcattatgttgtggaacaaagcgaatactcttattagctggtaattgagcgagttgaaaaaatcaagtctattggagggtatggtcagagtactgatagagatccctgttaagataatcgatctttttcaaatatccaatttcattccatcttgccatcgggtcttggcttcttacatcaataattaaaactacttactctattagtgccaaaaatggtaaaccgtattcaaattgctgcaagcatatgcttaaaaggatcgcgttgcgagcttcttttgagattcgcaagcttgattttatgctcttgtgggaagaaaagcaacccactgaattccagatttgttgtgttttcatgcatggacgacatactttgagtaataccgttactgagattttaccgaattcgcattgcgttgaggcgtgaagtttcttaatgctgtgccatatggttaagttgcgtttcaagatggtccacaagtatttttgtatttaagcagtgtcaattcaagcctaactgctcataaaaactacacggtttgctgatatcaaaaacgatgtttgagaagagtaaatttgtggtttcgtttctgcttttactccagctattttgtgtccttggtgtacatggagaaattgtcatgacccaaagtccatcaactctttctgcctcagttggtgatagagttatcattacttgtcagagttctcaatctgtgttcaacaattacttgagctggtaccaacaaaaacctggtagagcccccaaactgttaatctacgatgcatccaaactggctagcggagtaccttctaggtttagcggttccggatcaggtgcagaatttacactgacaatatcctctttgcaaccagacgactttgccacatactattgccaaggttcggattatagcggtggttgggactccgcgtttggtcaaggtaccaagttgactgttctcggtggaggtggaggttctggtggtggaggatcaggtggtggcggatctggcggtggagggtccgaggtgcagttggtagagtcgggcggtggatcagtccagcctggtggatccttgagactttcctgtaccgcttctggtatcgacttatccagttatcccatgtcgtgggttagacaagctccgggaaagggtttggaatgggttggtatcatcagcactagaggaaatacttactacgctacttgggctaagggacgttttacaattagtagagatacgtctaaaaacactgtgtatttgcagatgaattcactaagagccgaggacactgcaacttactactgtgcacgtggtctttacggtaataactattatggagctttcaatttgtggggacaaggcacaactgtaacggtgtcctcataataagcggccgcagcgaatttcttatgatttatgatttttattattaaataagttataaaaaaaataagtgtatacaaattttaaagtgactcttaggttttaaaacgaaaattcttattcttgagtaactctttcctgtaggtcaggttgctttctcaggtatagcatgaggtcgctcttattgaccacacctctaccggcatgccgagcaaatgcctgcaaatcgctccccatttcacccaattgtagatatgctaactccagcaatgagttgatgaatctcggtgtgtattttatgtcctcagaggacaaggatccttcagtaatgtcttgtttcttttgttgcagtggtgagccattttgacttcgtgaaagtttctttagaatagttgtttccagaggccaaacattccacccgtagtaaagtgcaagcgtaggaagaccaagactggcataaatcaggtataagtgtcgagcactggcaggtgatcttctgaaagtttctactagcagataagatccagtagtcatgcatatggcaacaatgtaccgtgtggatctaagaacgcgtcctactaaccttcgcattcgttggtccagtttgttgttatcgatcaacgtgacaaggttgtcgattccgcgtaagcatgcatacccaaggacgcctgttgcaattccaagtgagccagttccaacaatctttgtaatattagagcacttcattgtgttgcgcttgaaagtaaaatgcgaacaaattaagagataatctcgaaaccgcgacttcaaacgccaatatgatgtgcggcacacaataagcgttcatatccgctgggtgactttctcgctttaaaaaattatccgaaaaaattttctagagtgttgacactttatacttccggctcgtataatacgacaaggtgtaaggaggactaaaccatggctaaactcacctctgctgttccagtcctgactgctcgtgatgttgctggtgctgttgagttctggactgatagactcggtttctcccgtgacttcgtagaggacgactttgccggtgttgtacgtgacgacgttaccctgttcatctccgcagttcaggaccaggttgtgccagacaacactctggcatgggtatgggttcgtggtctggacgaactgtacgctgagtggtctgaggtcgtgtctaccaacttccgtgatgcatctggtccagctatgaccgagatcggtgaacagccctggggtcgtgagtttgcactgcgtgatccagctggtaactgcgtgcatttcgtcgcagaagagcaggactaacctctaggacaccttacgattatttagagagtatttattagttttattgtatgtatacggatgttttattatctatttatgcccttatattctgtaactatccaaaagtcctatcttatcaagccagcaatctatgtccgcgaacgtcaactaaaaataagctttttatgctcttctctctttttttcccttcggtataattataccttgcatccacagattctcctgccaaattttgcataatcctttacaacatggctatatgggagcacttagcgccctccaaaacccatattgcctacgcatgtataggtgttttttccacaatattttctctgtgctctctttttattaaagagaagctctatatcggagaagcttctgtggccgttatattcggccttatcgtgggaccacattgcctgaattggtttgccccggaagattggggaaacttggatctgattaccttagctgcaggtaccactgagcgtcagaccccgtagaaaagatcaaaggatcttcttgagatcctttttttctgcgcgtaatctgctgcttgcaaacaaaaaaaccaccgctaccagcggtggtttgtttgccggatcaagagctaccaactctttttccgaaggtaactggcttcagcagagcgcagataccaaatactgttcttctagtgtagccgtagttaggccaccacttcaagaactctgtagcaccgcctacatacctcgctctgctaatcctgttaccagtggctgctgccagtggcgataagtcgtgtcttaccgggttggactcaagacgatagttaccggataaggcgcagcggtcgggctgaacggggggttcgtgcacacagcccagcttggagcgaacgacctacaccgaactgagatacctacagcgtgagctatgagaaagcgccacgcttcccgaagggagaaaggcggacaggtatccggtaagcggcagggtcggaacaggagagcgcacgagggagcttccagggggaaacgcctggtatctttatagtcctgtcgggtttcgccacctctgacttgagcgtcgatttttgtgatgctcgtcaggggggcggagcctatggaaaaacgccagcaacgcggcctttttacggttcctggccttttgctggccttttgctcacatcg

SEQ ID NO: 4 - DNA, 9667 bp, Artificial Sequence
  synthetic vector sequence
cgatttattatgttacaatatggaagggaactttacacttctcctatgcacatatattaattaaagtccaatgctagtagagaaggggggtaacacccctccgcgctcttttccgatttttttctaaaccgtggaatatttcgcatatccttttgttgtttccgggtgtacaatatggacttcctcttttctggcaaccaaacccatacatcgggattcctataataccttcgttggtctccctaacatgtaggtggcggaggggagatatacaatagaacagataccagacaagacataatgggctaaacaagactacaccaattacactgcctcattgatggtggtacataacgaactaatactgtagccctagacttgatagccatcatcatatcgaagtttcactaccctttttccatttgccatctattgaagtaataataggcgcatgcaacttcttttctttttttttcttttctctctcccccgttgttgtctcaccatatccgcaatgacaaaaaaatgatggaagacactaaaggaaaaaattaacgacaaagacagcaccaacagatgtcgttgttccagagctgatgaggggtatctcgaagcacacgaaactttttccttccttcattcacgcacactactctctaatgagcaacggtatacggccttccttccagttacttgaatttgaaataaaaaaaagtttgctgtcttgctatcaagtataaatagacctgcaattattaatcttttgtttcctcgtcattgttctcgttccctttcttccttgtttctttttctgcacaatatttcaagctataccaagcatacaatcaactatctcatatacagtcgaccaaaacgatgaagtgggtcactttcatctcgctgctatttttgttctccagcgcctatagcgagattgtgatgactcaatccccttccactctaagcgcttctgtcggtgaccgtgttatcattacctgtcaatcctctcaatcggttttcaacaattacttatcctggtatcaacagaagccaggtcgtgcacctaaacttctgatttacgatgcttcaaaattggctagtggtgtcccaagcagattttcgggatctggttccggtgccgagtttacactcacgatctcctcacttcaacccgatgatttcgcaacatactattgtcaaggtagcgactatagtggaggttgggactctgcctttggacaaggtactaagctaacagttttgggtggaggcggaggttcgggtggtggtggatcaggaggaggtggtagtggcggaggaggctcagaagtgcaactggttgaaagtggtggaggttccgttcagccagggggttccttgagattgtcttgcactgcttctggtatcgacctgtcatcatacccaatgagctgggtaagacaggctcctggtaaaggtttggaatgggttggaattatctctactcgtggtaatacatattacgcaacatgggctaagggtagattcacaatatccagggatacttccaaaaacacagtatacttacaaatgaattctttgagagccgaggataccgctacctattactgtgcaaggggtctgtatggtaacaattactatggagcattcaatttgtggggtcagggcacgactgtgactgtcagctcataatagagatctccttttcctttgtccatatcatgtaattagttatgtcacgcttacattcacgccctccccccacatccgctctaaccgaaaaggaaggagttagacaacctgaagtctaggtccctatttatttttttatagttatgttagtattaagaacgttatttatatttcaaatttttcttttttttctgtacagacgcgtgtacgcatgtaacattatactgaaaaccttgcttgagaaggttttgggacgctcgaaggctttaatttgcaagctgccgtatgggctttttgtagaaatgtcttggtgtcctcgtccaatcaggtagccatctctgaaatatctggctccgttgcaactccgaacgacctgctggcaacgtaaaattctccggggtaaaacttaaatgtggagtaatggaaccagaaacgtctcttcccttctctctccttccaccgcccgttaccgtcactaggaaattttactctgctggagagcttcttctacggcccccttgcagcaatgctcttcccagcattacgttgcgggtaaaacggaggtcgtgtacccgacctagcagcccagggatggaaaagtcccggccgtcgctggcaataatagcgggcggacgcatgtcatgagattattggaaaccaccagaatcgaatataaaaggcgaacacctttcccaattttggtttctcctgacccaaagactttaaatttaatttatttgtccctatttcaatcaattgaacaactatcaaaacacactcgagcaaaacgatgcgtttcccatcgattttcacagctgttctgtttgcagcttcatctgctttagctgcacctgttaacacaactacagaggacgaaacggcccagatcccagctgaggcagtcattggttattccgatttggaaggtgatttcgatgtcgctgtgttaccattcagtaattccacaaataacggtttgctgttcattaacaccactatagcaagcatcgctgcaaaagaggaaggtgtttccctagaaaagagggagattgttatgacgcagtcccccagtactttgtctgcttccgttggagatagagtaatcataacttgtcaatcctctcaatctgtctttaacaattacctttcttggtaccaacagaaaccaggcagggctccaaagttgctaatctatgatgcatctaaactggcctccggtgttccatcacgtttttcaggttcaggatccggtgctgagttcactttaacgatttcctcgttgcaaccggatgactttgccacatattactgtcaaggttctgactactcaggtggttgggactctgctttcggtcaaggtaccaaactgactgtattgggaggaggtggaggtagcggcggtggaggttcaggaggtggtggatccggagggggtggaagtgaagttcaattggtggaaagcggtggtggttccgttcagcctggaggtagcttgcgtctgtcgtgcactgcaagtggtattgacttaagctcatatcctatgtcttgggtcagacaagcacctggtaagggtttggagtgggtcggcatcattagcactagaggtaacacatactatgctacatgggcaaagggaagattcacaatctcacgtgatacatctaaaaatacagtttatcttcagatgaatagtctcagagctgaagatacagctacctactactgtgccagaggattatacggtaataactattatggtgcattcaatctatggggccaaggtactactgtgaccgtgtcctcgtaatagaggccttgttctttcctgcggtacccagatccaattcccgctttgactgcctgaaatctccatcgcctacaatgatgacatttggatttggttgactcatgttggtattgtgaaatagacgcagatcgggaacactgaaaaatacacagttattattcatttaaatcacggtcttggagtcatcaggctctgactgggcagctgctgcaactggaacttcccaagcctcccaccaaacagcaggtgtagccgaaagtattcacgtgtcccagaatgaggcccacagtacatctgtcaccgtttctcaacccccttcaacggtttctttgcaaattggagaagcaaataccctgaaatggtcagctttctttggagtagtagttccgctgctcaacgtactcttcgtttaaaagccctcctaggacaaaatggccaagctgggaaacgggatttggtggaactttattattctttctacgatccaagcattatgttgtggaacaaagcgaatactcttattagctggtaattgagcgagttgaaaaaatcaagtctattggagggtatggtcagagtactgatagagatccctgttaagataatcgatctttttcaaatatccaatttcattccatcttgccatcgggtcttggcttcttacatcaataattaaaactacttactctattagtgccaaaaatggtaaaccgtattcaaattgctgcaagcatatgcttaaaaggatcgcgttgcgagcttcttttgagattcgcaagcttgattttatgctcttgtgggaagaaaagcaacccactgaattccagatttgttgtgttttcatgcatggacgacatactttgagtaataccgttactgagattttaccgaattcgcattgcgttgaggcgtgaagtttcttaatgctgtgccatatggttaagttgcgtttcaagatggtccacaagtatttttgtatttaagcagtgtcaattcaagcctaactgctcataaaaactacacggtttgctgatatcaaaaacgatgtttgagaagagtaaatttgtggtttcgtttctgcttttactccagctattttgtgtccttggtgtacatggagaaattgtcatgacccaaagtccatcaactctttctgcctcagttggtgatagagttatcattacttgtcagagttctcaatctgtgttcaacaattacttgagctggtaccaacaaaaacctggtagagcccccaaactgttaatctacgatgcatccaaactggctagcggagtaccttctaggtttagcggttccggatcaggtgcagaatttacactgacaatatcctctttgcaaccagacgactttgccacatactattgccaaggttcggattatagcggtggttgggactccgcgtttggtcaaggtaccaagttgactgttctcggtggaggtggaggttctggtggtggaggatcaggtggtggcggatctggcggtggagggtccgaggtgcagttggtagagtcgggcggtggatcagtccagcctggtggatccttgagactttcctgtaccgcttctggtatcgacttatccagttatcccatgtcgtgggttagacaagctccgggaaagggtttggaatgggttggtatcatcagcactagaggaaatacttactacgctacttgggctaagggacgttttacaattagtagagatacgtctaaaaacactgtgtatttgcagatgaattcactaagagccgaggacactgcaacttactactgtgcacgtggtctttacggtaataactattatggagctttcaatttgtggggacaaggcacaactgtaacggtgtcctcataataagcggccgcagcgaatttcttatgatttatgatttttattattaaataagttataaaaaaaataagtgtatacaaattttaaagtgactcttaggttttaaaacgaaaattcttattcttgagtaactctttcctgtaggtcaggttgctttctcaggtatagcatgaggtcgctcttattgaccacacctctaccggcatgccgagcaaatgcctgcaaatcgctccccatttcacccaattgtagatatgctaactccagcaatgagttgatgaatctcggtgtgtattttatgtcctcagaggacaaggatcccttgccaacagggagttcttcagagacatggaggctcaaaacgaaattattgacagcctagacatcaatagtcatacaacagaaagcgaccacccaactttggctgataatagcgtataaacaatgcatactttgtacgttcaaaatacaatgcagtagatatatttatgcatattacatataatacatatcacataggaagcaacaggcgcgttggacttttaattttcgaggaccgcgaatccttacatcacacccaatcccccacaagtgatcccccacacaccatagcttcaaaatgtttctactccttttttactcttccagattttctcggactccgcgcatcgccgtaccacttcaaaacacccaagcacagcatactaaatttcccctctttcttcctctagggtgtcgttaattacccgtactaaaggtttggaaaagaaaaaagagaccgcctcgtttctttttcttcgtcgaaaaaggcaataaaaatttttatcacgtttctttttcttgaaaatttttttttttgatttttttctctttcgatgacctcccattgatatttaagttaataaacggtcttcaatttctcaagtttcagtttcatttttcttgttctattacaactttttttacttcttgctcattagaaagaaagcatagcaatctaatctaagttttaattacaaaactagtcaaaacgatgagatttccttcaatttttactgctgttttattcgcagcatcctccgcattagctgaaattgtcatgacccaaagcccatccactctgtctgcttccgttggtgaccgtgttatcataacatgtcagtcaagccaatcggttttcaataactatctatcatggtatcaacaaaaacctggacgtgcaccaaagttacttatctacgatgctagtaaactggcaagtggagtaccttcgagattcagcggctccggttctggtgctgaattcacattgacgatttccagtctacaaccagatgactttgctacttactactgccaaggttcagactattccggaggatgggactccgcatttggtcagggaacaaaattgactgtgttaggtgggggcggaggtagcggtggaggtggttcgggaggtggcggttccggtggtggtggttccgaagtgcagttggttgagtctggtggaggttctgtccaacccggaggatcccttagattgtcatgtacagcctctggtattgatttgtctagttacccaatgtcatgggttaggcaggcccctggtaagggactggagtgggtaggtattatctcaactagaggcaatacttattacgcaacgtgggcaaagggtagatttaccatctctagggatacctccaaaaacacagtctatctgcaaatgaatagcttgagagctgaggatactgctacatattactgtgcccgtggattgtatggtaacaattactacggtgctttcaatctctggggtcaaggtacaactgtgactgtttcatcttaataggagctctcaagaggatgtcagaatgccatttgcctgagagatgcaggcttcatttttgatacttttttatttgtaacctatatagtataggattttttttgtcattttgtttcttctcgtacgagcttgctcctgatcagcctatctcgcagcagatgaatatcttgtggtaggggtttgggaaaatcattcgagtttgatgtttttcttggtatttcccactcctcttcagagtacagaagattaagtgagaccttcgtttgtgccttcagtaatgtcttgtttcttttgttgcagtggtgagccattttgacttcgtgaaagtttctttagaatagttgtttccagaggccaaacattccacccgtagtaaagtgcaagcgtaggaagaccaagactggcataaatcaggtataagtgtcgagcactggcaggtgatcttctgaaagtttctactagcagataagatccagtagtcatgcatatggcaacaatgtaccgtgtggatctaagaacgcgtcctactaaccttcgcattcgttggtccagtttgttgttatcgatcaacgtgacaaggttgtcgattccgcgtaagcatgcatacccaaggacgcctgttgcaattccaagtgagccagttccaacaatctttgtaatattagagcacttcattgtgttgcgcttgaaagtaaaatgcgaacaaattaagagataatctcgaaaccgcgacttcaaacgccaatatgatgtgcggcacacaataagcgttcatatccgctgggtgactttctcgctttaaaaaattatccgaaaaaattttctagagtgttgacactttatacttccggctcgtataatacgacaaggtgtaaggaggactaaaccatggctaaactcacctctgctgttccagtcctgactgctcgtgatgttgctggtgctgttgagttctggactgatagactcggtttctcccgtgacttcgtagaggacgactttgccggtgttgtacgtgacgacgttaccctgttcatctccgcagttcaggaccaggttgtgccagacaacactctggcatgggtatgggttcgtggtctggacgaactgtacgctgagtggtctgaggtcgtgtctaccaacttccgtgatgcatctggtccagctatgaccgagatcggtgaacagccctggggtcgtgagtttgcactgcgtgatccagctggtaactgcgtgcatttcgtcgcagaagagcaggactaacctctaggacaccttacgattatttagagagtatttattagttttattgtatgtatacggatgttttattatctatttatgcccttatattctgtaactatccaaaagtcctatcttatcaagccagcaatctatgtccgcgaacgtcaactaaaaataagctttttatgctcttctctctttttttcccttcggtataattataccttgcatccacagattctcctgccaaattttgcataatcctttacaacatggctatatgggagcacttagcgccctccaaaacccatattgcctacgcatgtataggtgttttttccacaatattttctctgtgctctctttttattaaagagaagctctatatcggagaagcttctgtggccgttatattcggccttatcgtgggaccacattgcctgaattggtttgccccggaagattggggaaacttggatctgattaccttagctgcaggtaccactgagcgtcagaccccgtagaaaagatcaaaggatcttcttgagatcctttttttctgcgcgtaatctgctgcttgcaaacaaaaaaaccaccgctaccagcggtggtttgtttgccggatcaagagctaccaactctttttccgaaggtaactggcttcagcagagcgcagataccaaatactgttcttctagtgtagccgtagttaggccaccacttcaagaactctgtagcaccgcctacatacctcgctctgctaatcctgttaccagtggctgctgccagtggcgataagtcgtgtcttaccgggttggactcaagacgatagttaccggataaggcgcagcggtcgggctgaacggggggttcgtgcacacagcccagcttggagcgaacgacctacaccgaactgagatacctacagcgtgagctatgagaaagcgccacgcttcccgaagggagaaaggcggacaggtatccggtaagcggcagggtcggaacaggagagcgcacgagggagcttccagggggaaacgcctggtatctttatagtcctgtcgggtttcgccacctctgacttgagcgtcgatttttgtgatgctcgtcaggggggcggagcctatggaaaaacgccagcaacgcggcctttttacggttcctggccttttgctggccttttgctcacatcg

SEQ ID NO: 5 - DNA, 9456 bp, Artificial Sequence
  synthetic vector sequence
aattcggatctaataaaatatctttattttcattacatctgtgtgttggttttttgtgtggatcttcaatattggccattagccatattattcattggttatatagcataaatcaatattggctattggccattgcatacgttgtatctatatcataatatgtacatttatattggctcatgtccaatatgaccgccatgttggcattgattattgactagttattaatagtaatcaattacggggtcattagttcatagcccatatatggagttccgcgttacataacttacggtaaatggcccgcctggctgaccgcccaacgacccccgcccattgacgtcaataatgacgtatgttcccatagtaacgccaatagggactttccattgacgtcaatgggtggagtatttacggtaaactgcccacttggcagtacatcaagtgtatcatatgccaagtacgccccctattgacgtcaatgacggtaaatggcccgcctggcattatgcccagtacatgaccttatgggactttcctacttggcagtacatctacgtattagtcatcgctattaccatggtgatgcggttttggcagtacatcaatgggcgtggatagcggtttgactcacggggatttccaagtctccaccccattgacgtcaatgggagtttgttttggcaccaaaatcaacgggactttccaaaatgtcgtaacaactccgccccattgacgcaaatgggcggtaggcgtgtacggtgggaggtctatataagcagagctcgtttagtgaaccgtcagatcgcctggagacgccatccacgctgttttgacctccatagaagacaccgggaccgatccagcctccgcggccgggaacggtgcattggaacgcggattccccgtgccaagagtgacgtaagtaccgcctatagagtctataggcccacccccttggcttcgttagaacgcggctacaattaatacataaccttatgtatcatacacatacgatttaggtgacactatagaataacatccactttgcctttctctccacaggtgtccactcccaggtccaactgcacctcggttctatcgaaaacgcgcctctagacctgcaggccaccatggcccccgtggccgtgtgggccgccctggccgtgggcctggagctgtgggccgccgcccacgccctgcccgcccaggtggccttcaccccctacgcccccgagcccggctccacctgccggctgcgggagtactacgaccagaccgcccagatgtgctgctccaagtgctcccccggccagcacgccaaggtgttctgcaccaagacctccgacaccgtgtgcgactcctgcgaggactccacctacacccagctgtggaactgggtgcccgagtgcctgtcctgcggctcccggtgctcctccgaccaggtggagacccaggcctgcacccgggagcagaaccggatctgcacctgccggcccggctggtactgcgccctgtccaagcaggagggctgccggctgtgcgcccccctgcggaagtgccggcccggcttcggcgtggcccggcccggcaccgagacctccgacgtggtgtgcaagccctgcgcccccggcaccttctccaacaccacctcctccaccgacatctgccggccccaccagatctgcaacgtggtggccatccccggcaacgcctccatggacgccgtgtgcacctccacctcccccacccggtccatggcccccggcgccgtgcacctgccccagcccgtgtccacccggtcccagcacacccagcccacccccgagccctccaccgccccctccacctccttcctgctgcccatgggcccctccccccccgccgagggctccaccggcgacgagcccaagtcctgcgacaagacccacacctgccccccctgccccgcccccgagctgctgggcggcccctccgtgttcctgttcccccccaagcccaaggacaccctgatgatctcccggacccccgaggtgacctgcgtggtggtggacgtgtcccacgaggaccccgaggtgaagttcaactggtacgtggacggcgtggaggtgcacaacgccaagaccaagccccgggaggagcagtacaactccacctaccgggtggtgtccgtgctgaccgtgctgcaccaggactggctgaacggcaaggagtacaagtgcaaggtgtccaacaaggccctgcccgcccccatcgagaagaccatctccaaggccaagggccagccccgggagccccaggtgtacaccctgcccccctcccgggaggagatgaccaagaaccaggtgtccctgacctgcctggtgaagggcttctacccctccgacatcgccgtggagtgggagtccaacggccagcccgagaacaactacaagaccaccccccccgtgctggactccgacggctccttcttcctgtactccaagctgaccgtggacaagtcccggtggcagcagggcaacgtgttctcctgctccgtgatgcacgaggccctgcacaaccactacacccagaagtccctgtccctgtcccccggcaagtgatgaggcgcgcccctagagtcgacccgggcggccgcttccctttagtgagggttaatgcttcgagcgactgtgccttctagttgccagccatctgttgtttgcccctcccccgtgccttccttgaccctggaaggtgccactcccactgtcctttcctaataaaatgaggaaattgcatcgcattgtctgagtaggtgtcattctattctggggggtggggtggggcaggacagcaagggggaggattgggaagacaatagcaggcatgctggggatgcggtgggctctatggaaatccgataaggatcgatccgggctggcgtaatagcgaagaggcccgcaccgatcgcccttcccaacagttgcgcagcctgaatggcgaatggacgcgccctgtagcggcgcattaagcgcggcgggtgtggtggttacgcgcagcgtgaccgctacacttgccagcgccctagcgcccgctcctttcgctttcttcccttcctttctcgccacgttcgccggctttccccgtcaagctctaaatcgggggctccctttagggttccgatttagagctttacggcacctcgaccgcaaaaaacttgatttgggtgatggttcacgtagtgggccatcgccctgatagacggtttttcgccctttgacgttggagtccacgttctttaatagtggactcttgttccaaactggaacaacactcaaccctatctcggtctattcttttgatttataagggattttgccgatttcggcctattggttaaaaaatgagctgatttaacaaatatttaacgcgaattttaacaaaatattaacgtttacaatttcgcctgatgcggtattttctccttacgcatctgtgcggtatttcacaccgcatacgcggatctttggggttgcgccttttccaaggcagccctgggtttgcgcagggacgcggctgctctgggcgtggttccgggaaacgcagcggcgccgaccctgggtctcgcacattcttcacgtccgttcgcagcgtcacccggatcttcgccgctacccttgtgggccccccggcgacgcttcctgctccgcccctaagtcgggaaggttccttgcggttcgcggcgtgccggacgtgacaaacggaagccgcacgtctcactagtaccctcgcagacggacagcgccagggagcaatggcagcgcgccgaccgcgatgggctgtggccaatagcggctgctcagcagggcgcgccgagagcagcggccgggaaggggcggtgcgggaggcggggtgtggggcggtagtgtgggccctgttcctgcccgcgcggtgttccgcattctgcaagcctccggagcgcacgtcggcagtcggctccctcgttgaccgaatcaccgacctctctccccagggggatccaccggagcttaccatgaccgagtacaagcccacggtgcgcgctagcgctaccggtcgccaccatgattgaacaagatggattgcacgcaggttctccggccgcttgggtggagaggctattcggctatgactgggcacaacagacaatcggctgctctgatgccgccgtgttccggctgtcagcgcaggggcgcccggttctttttgtcaagaccgacctgtccggtgccctgaatgaactgcaggacgaggcagcgcggctatcgtggctggccacgacgggcgttccttgcgcagctgtgctcgacgttgtcactgaagcgggaagggactggctgctattgggcgaagtgccggggcaggatctcctgtcatctcaccttgctcctgccgagaaagtatccatcatggctgatgcaatgcggcggctgcatacgcttgatccggctacctgcccattcgaccaccaagcgaaacatcgcatcgagcgagcacgtactcggatggaagccggtcttgtcgatcaggatgatctggacgaagagcatcaggggctcgcgccagccgaactgttcgccaggctcaaggcgcgcatgcccgacggcgaggatctcgtcgtgacccatggcgatgcctgcttgccgaatatcatggtggaaaatggccgcttttctggattcatcgactgtggccggctgggtgtggcggaccgctatcaggacatagcgttggctacccgtgatattgctgaagagcttggcggcgaatgggctgaccgcttcctcgtgctttacggtatcgccgctcccgattcgcagcgcatcgccttctatcgccttcttgacgagttcttctgagcgggactctggggttcgaaatgaccgaccaagcgacgcccaacctgccatcacgatggccgcgatgagtcgacccgggcggccgcttccctttagtgagggttaatgcttcgagactcctcaggtgcaggctgcctatcagaaggtggtggctggtgtggccaatgccctggctcacaaataccactgagatctttttccctctgccaaaaattatggggacatcatgaagccccttgagcatctgacttctggctaataaaggaaatttattttcattgcaatagtgtgttggaattttttgtgtctctcactcggaaggacatatgggagggcaaatcatttaaaacatcagaatgagtatttggtttagagtttggcaacatatgcccatatgctggctgccatgaacaaaggttggctataaagaggtcatcagtatatgaaacagccccctgctgtccattccttattccatagaaaagccttgacttgaggttagattttttttatattttgttttgtgttatttttttctttaacatccctaaaattttccttacatgttttactagccagatttttcctcctctcctgactactcccagtcatagctgtccctcttctcttatggagatccctcgacaatcgatagcgataaggatccgcgtatggtgcactctcagtacaatctgctctgatgccgcatagttaagccagccccgacacccgccaacacccgctgacgcgccctgacgggcttgtctgctcccggcatccgcttacagacaagctgtgaccgtctccgggagctgcatgtgtcagaggttttcaccgtcatcaccgaaacgcgcgagacgaaagggcctcgtgatacgcctatttttataggttaatgtcatgataataatggtttcttagacgtcaggtggcacttttcggggaaatgtgcgcggaacccctatttgtttatttttctaaatacattcaaatatgtatccgcttaccaatgcttaatcagtgaggcacctatctcagcgatctgtctatttcgttcatccatagttgcctgactccccgtcgtgtagataactacgatacgggagggcttaccatctggccccagtgctgcaatgataccgcgggacccacgctcaccggctccagatttatcagcaataaaccagccagccggaagggccgagcgcagaagtggtcctgcaactttatccgcctccatccagtctattaattgttgccgggaagctagagtaagtagttcgccagttaatagtttgcgcaacgttgttgccattgctacaggcatcgtggtgtcacgctcgtcgtttggtatggcttcattcagctccggttcccaacgatcaaggcgagttacatgatcccccatgttgtgcaaaaaagcggttagctccttcggtcctccgatcgttgtcagaagtaagttggccgcagtgttatcactcatggttatggcagcactgcataattctcttactgtcatgccatccgtaagatgcttttctgtgactggtgagtactcaaccaagtcattctgagaatagtgtatgcggcgaccgagttgctcttgcccggcgtcaatacgggataataccgcgccacatagcagaactttaaaagtgctcatcattggaaaacgttcttcggggcgaaaactctcaaggatcttaccgctgttgagatccagttcgatgtaacccactcgtgcacccaactgatcttcagcatcttttactttcaccagcgtttctgggtgagcaaaaacaggaaggcaaaatgccgcaaaaaagggaataagggcgacacggaaatgttgaatactcatactcttcctttttcaatattattgaagcatttatcagggttattgtctcatgagcggatacatatttgaatgtatttagaaaaataaacaaataggggttccgcgcacatttccccgaaaagtgccacctgtcatgaccaaaatcccttaacgtgagttttcgttccactgagcgtcagaccccgtagaaaagatcaaaggatcttcttgagatcctttttttctgcgcgtaatctgctgcttgcaaacaaaaaaaccaccgctaccagcggtggtttgtttgccggatcaagagctaccaactctttttccgaaggtaactggcttcagcagagcgcagataccaaatactgttcttctagtgtagccgtagttaggccaccacttcaagaactctgtagcaccgcctacatacctcgctctgctaatcctgttaccagtggctgctgccagtggcgataagtcgtgtcttaccgggttggactcaagacgatagttaccggataaggcgcagcggtcgggctgaacggggggttcgtgcacacagcccagcttggagcgaacgacctacaccgaactgagatacctacagcgtgagctatgagaaagcgccacgcttcccgaagggagaaaggcggacaggtatccggtaagcggcagggtcggaacaggagagcgcacgagggagcttccagggggaaacgcctggtatctttatagtcctgtcgggtttcgccacctctgacttgagcgtcgatttttgtgatgctcgtcaggggggcggagcctatggaaaaacgccagcaacgcgggctcgacagatccatttaaattttcaccgtcatcaccgaaacgcgcgaggcagctgtggaatgtgtgtcagttagggtgtggaaagtccccaggctccccagcaggcagaagtatgcaaagcatgcatctcaattagtcagcaaccaggtgtggaaagtccccaggctccccagcaggcagaagtatgcaaagcatgcatctcaattagtcagcaaccatagtcccgcccctaactccgcccatcccgcccctaactccgcccagttccgcccattctccgccccatggctgactaattttttttatttatgcagaggccgaggccgcctcggccctctgagctattccagaagtagtgaggaggcttttttggaggcctaggcttttgcaaaaagctaattcgagctcggtacccccaaacttgacggcaatcctagcgtgaaggctggtaggattttatccccgctgccatcatggttcgaccattgaactgcatcgtcgccgtgtcccaaaatatggggattggcaagaacggagaccgaccctggcctccgctcaggaacgagttcaagtacttccaaagaatgaccacaacctcttcagtggaaggtaaacagaatctggtgattatgggtaggaaaacctggttctccattcctgagaagaatcgacctttaaaggacagaattaatatagttctcagtagagaactcaaagaaccaccacgaggagctcattttcttgccaaaagtttggatgatgccttaagacttattgaacaaccggaattggcaagtaaagtagacatggtttggatagtcggaggcagttctgtttaccaggaagccatgaatcaaccaggccacctcagactctttgtgacaaggatcatgcaggaatttgaaagtgacacgtttttcccagaaattgatttggggaaatataaacttctcccagaatacccaggcgtcctctctgaggtccaggaggaaaaaggcatcaagtataagtttgaagtctacgagaagaaagactaacaggaagatgctttcaagttctctgctcccctcctaaagctatgcatttttataagaccatgggggatgctcgatcccctcgcgagttggttcagctgctgcctgaggctggacgacctcgcggagttctaccggcagtgcaaatccgtcggcatccaggaaaccagcagcggctatccgcgcatccatgcccccgaactgcaggagtggggaggcacgatggccgctttggtccggatctttgtgaaggaaccttacttctgtggtgtgacataattggacaaactacctacagagatttaaagctctaaggtaaatataaaatttttaagtgtataatgtgttaaactactgattctaattgtttgtgtattttagattccaacctatggaactgatgaatgggagcagtggtggaatgcctttaatgaggaaaacctgttttgctcagaagaaatgccatctagtgatgatgaggctactgctgactctcaacattctactcctccaaaaaagaagagaaaggtagaagaccccaaggactttccttcagaattgctaagttttttgagtcatgctgtgtttagtaatagaactcttgcttgctttgctatttacaccacaaaggaaaaagctgcactgctatacaagaaaattatggaaaaatattctgtaacctttataagtaggcataacagttataatcataacatactgttttttcttactccacacaggcatagagtgtctgctattaataactatgctcaaaaattgtgtacctttagctttttaatttgtaaaggggttaataaggaatatttgatgtatagtgccttgactagagatcataatcagccag

SEQ ID NO: 6 - DNA, 10783 bp, Artificial Sequence
  synthetic vector sequence
aattcggatctgcgcagcaccatggcctgaaataacctctgaaagaggaacttggttaggtaccttctgaggcggaaagaaccagctgtggaatgtgtgtcagttagggtgtggaaagtccccaggctccccagcaggcagaagtatgcaaagcatgcatctcaattagtcagcaaccaggtgtggaaagtccccaggctccccagcaggcagaagtatgcaaagcatgcatctcaattagtcagcaaccatagtcccgcccctaactccgcccatcccgcccctaactccgcccagttccgcccattctccgccccatggctgactaattttttttatttatgcagaggccgaggccgcctcggcctctgagctattccagaagtagtgaggaggcttttttggaggcctaggcttttgcaaaaagcttctcgaggaacttcagggtgagtctatgggacccttgatgttttctttccccttcttttctatggttaagttcatgtcataggaaggggagaagtaacagggtacagtttagaatgggaaacagacgaatgattgcatcagtgtggaagtctcaggatcgttttagtttcttttatttgctgttcataacaattgttttcttttgtttaattcttgctttctttttttttcttctccgcaatttttactattatacttaatgccttaacattgtgtataacaaaaggaaatatctctgagatacattaagtaacttaaaaaaaaactttacacagtctgcctagtacattactatttggaatatatgtgtgcttatttgcatattcataatctccctactttattttcttttatttttaattgatacataatcattatacatatttatgggttaaagtgtaatgttttaatatgtgtacacatattgaccaaatcagggtaattttgcatttgtaattttaaaaaatgctttcttcttttaatatacttttttgtttatcttatttctaatactttccctaatctctttctttcagggcaataatgatacaatgtatcatgcctctttgcaccattctaaagaataacagtgataatttctgggttaaggcaatagcaatatttctgcatataaatatttctgcatataaattgtaactgatgtaagaggtttcatattgctaatagcagctacaatccagctaccattctgcttttattttatggttgggataaggctggattattctgagtccaagctaggcccttttgctaatcatgttcatacctcttatcttcctcccacagctcctgggcagtgtccactcccaggtccaactgcacctcggttctatcgaaaacgcgtccaccatgaagtgggtgaccttcatctccctgctgttcctgttctcctccgcctactccctgcccgcccaggtggccttcaccccctacgcccccgagcccggctccacctgccggctgcgggagtactacgaccagaccgcccagatgtgctgctccaagtgctcccccggccagcacgccaaggtgttctgcaccaagacctccgacaccgtgtgcgactcctgcgaggactccacctacacccagctgtggaactgggtgcccgagtgcctgtcctgcggctcccggtgctcctccgaccaggtggagacccaggcctgcacccgggagcagaaccggatctgcacctgccggcccggctggtactgcgccctgtccaagcaggagggctgccggctgtgcgcccccctgcggaagtgccggcccggcttcggcgtggcccggcccggcaccgagacctccgacgtggtgtgcaagccctgcgcccccggcaccttctccaacaccacctcctccaccgacatctgccggccccaccagatctgcaacgtggtggccatccccggcaacgcctccatggacgccgtgtgcacctccacctcccccacccggtccatggcccccggcgccgtgcacctgccccagcccgtgtccacccggtcccagcacacccagcccacccccgagccctccaccgccccctccacctccttcctgctgcccatgggcccctccccccccgccgagggctccaccggcgacgagcccaagtcctgcgacaagacccacacctgccccccctgccccgcccccgagctgctgggcggcccctccgtgttcctgttcccccccaagcccaaggacaccctgatgatctcccggacccccgaggtgacctgcgtggtggtggacgtgtcccacgaggaccccgaggtgaagttcaactggtacgtggacggcgtggaggtgcacaacgccaagaccaagccccgggaggagcagtacaactccacctaccgggtggtgtccgtgctgaccgtgctgcaccaggactggctgaacggcaaggagtacaagtgcaaggtgtccaacaaggccctgcccgcccccatcgagaagaccatctccaaggccaagggccagccccgggagccccaggtgtacaccctgcccccctcccgggaggagatgaccaagaaccaggtgtccctgacctgcctggtgaagggcttctacccctccgacatcgccgtggagtgggagtccaacggccagcccgagaacaactacaagaccaccccccccgtgctggactccgacggctccttcttcctgtactccaagctgaccgtggacaagtcccggtggcagcagggcaacgtgttctcctgctccgtgatgcacgaggccctgcacaaccactacacccagaagtccctgtccctgtcccccggcaagtgatgaggcgcgcccctagagtcgacccgggcggccgcttccctttagtgagggttaatgcttcgagcagacatgataagatacattgatgagtttggacaaaccacaactagaatgcagtgaaaaaaatgctttatttgtgaaatttgtgatgctattgctttatttgtaaccattataagctgcaataaacaagttaacaacaacaattgcattcattttatgtttcaggttcagggggagatgtgggaggttttttaaagcaagtaaaacctctacaaatgtggtaaaatccgataaggatcgatccgggctggcgtaatagcgaagaggcccgcaccgatcgcccttcccaacagttgcgcagcctgaatggcgaatggaacgcgccctgtagcggcgcattaagcgcggcgggtgtggtggttacgcgcagcgtgaccgctacacttgccagcgccctagcgcccgctcctttcgctttcttcccttcctttctcgccacgttcgccggctttccccgtcaagctctaaatcgggggctccctttagggttccgatttagagctttacggcacctcgaccgcaaaaaacttgatttgggtgatggttcacgtagtgggccatcgccctgatagacggtttttcgccctttgacgttggagtccacgttctttaatagtggactcttgttccaaactggaacaacactcaaccctatctcggtctattcttttgatttataagggattttgccgatttcggcctattggttaaaaaatgagctgatttaacaaatatttaacgcgaattttaacaaaatattaacgtttacaatttcgcctgatgcggtattttctccttacgcatctgtgcggtatttcacaccgcatacgcggatctgctttgcttctcaatttcttatttgcataatgagaaaaaaaggaaaattaattttaacaccaattcagtagttgattgagcaaatgcgttgccaaaaaggatgctttagagacagtgttctctgcacagataaggacaaacattattcagagggagtacccagagctgagactcctaagccagtgagtggcacagcattctagggagaaatatgcttgtcatcaccgaagcctgattccgtagagccacaccttggtaagggccaatctgctcacacaggatagagagggcaggagccagggcagagcatataaggtgaggtaggatcagttgctcctcacatttgcttctgacatagttgtgttggctagcgctaccggtcgccaccatgattgaacaagatggattgcacgcaggttctccggccgcttgggtggagaggctattcggctatgactgggcacaacagacaatcggctgctctgatgccgccgtgttccggctgtcagcgcaggggcgcccggttctttttgtcaagaccgacctgtccggtgccctgaatgaactgcaggacgaggcagcgcggctatcgtggctggccacgacgggcgttccttgcgcagctgtgctcgacgttgtcactgaagcgggaagggactggctgctattgggcgaagtgccggggcaggatctcctgtcatctcaccttgctcctgccgagaaagtatccatcatggctgatgcaatgcggcggctgcatacgcttgatccggctacctgcccattcgaccaccaagcgaaacatcgcatcgagcgagcacgtactcggatggaagccggtcttgtcgatcaggatgatctggacgaagagcatcaggggctcgcgccagccgaactgttcgccaggctcaaggcgcgcatgcccgacggcgaggatctcgtcgtgacccatggcgatgcctgcttgccgaatatcatggtggaaaatggccgcttttctggattcatcgactgtggccggctgggtgtggcggaccgctatcaggacatagcgttggctacccgtgatattgctgaagagcttggcggcgaatgggctgaccgcttcctcgtgctttacggtatcgccgctcccgattcgcagcgcatcgccttctatcgccttcttgacgagttcttctgacgactgtgccttctagttgccagccatctgttgtttgcccctcccccgtgccttccttgaccctggaaggtgccactcccactgtcctttcctaataaaatgaggaaattgcatcgcattgtctgagtaggtgtcattctattctggggggtggggtggggcaggacagcaagggggaggattgggaagacaatagcaggcatgctggggatgcggtgggctctatggaatcgatagcgataaggatccgcgtatggtgcactctcggttgccgccgggcgttttttattggtgagaatccaagctagaggcatcaaataaaacgaaaggctcagtcgaaagactgggcctttcgttttatctgttgtttgtcggtgaacgctctcctgagtaggacaaatccgccgccctagacctagggatatattccgcttcctcgctcactgactcgctacgctcggtcgttcgactgcggcgagcggaaatggcttacgaacggggcggagatttcctggaagatgccaggaagatacttaacagggaagtgagagggccgcggcaaagccgtttttccataggctccgcccccctgacaagcatcacgaaatctgacgctcaaatcagtggtggcgaaacccgacaggactataaagataccaggcgtttccccctggcggctccctcgtgcgctctcctgttcctgcctttcggtttaccggtgtcattccgctgttatggccgcgtttgtctcattccacgcctgacactcagttccgggtaggcagttcgctccaagctggactgtatgcacgaaccccccgttcagtccgaccgctgcgccttatccggtaactatcgtcttgagtccaacccggaaagacatgcaaaagcaccactggcagcagccactggtaattgatttagaggagttagtcttgaagtcatgcgccggttaaggctaaactgaaaggacaagttttggtgactgcgctcctccaagccagttacctcggttcaaagagttggtagctcagagaaccttcgaaaaaccgccctgcaaggcggttttttcgttttcagagcaagagattacgcgcagaccaaaacgatctcaagaagatcatcttattaatcagataaaatatttctagatttcagtgcaatttatctcttcaaatgtagcacctgaagtcagccccatacgatataagttgttactagtgcttggattctcaccaataaaaaacgcccggcggcaaccgagcgttctgaacaaatccagatggagttctgaggtcattactggatctatcaacaggagtccaagcgagctcgatatccgtcggcttgaacgaattgttagacattatttgccgactaccttggtgatctcgcctttcacgtagtggacaaattcttccaactgatctgcgcgcgaggccaagcgatcttcttcttgtccaagataagcctgtctagcttcaagtatgacgggctgatactgggccggcaggcgctccattgcccagtcggcagcgacatccttcggcgcgattttgccggttactgcgctgtaccaaatgcgggacaacgtaagcactacatttcgctcatcgccagcccagtcgggcggcgagttccatagcgttaaggtttcatttagcgcctcaaatagatcctgttcaggaaccggatcaaagagttcctccgccgctggacctaccaaggcaacgctatgttctcttgcttttgtcagcaagatagccagatcaatgtcgatcgtggctggctcgaagatacctgcaagaatgtcattgcgctgccattctccaaattgcagttcgcgcttagctggataacgccacggaatgatgtcgtcgtgcacaacaatggtgacttctacagcgcggagaatctcgctctctccaggggaagccgaagtttccaaaaggtcgttgatcaaagctcgccgcgttgtttcatcaagccttacggtcaccgtaaccagcaaatcaatatcactgtgtggcttcaggccgccatccactgcggagccgtacaaatgtacggccagcaacgtcggttcgagatggcgctcgatgacgccaactacctctgatagttgagtcgatacttcggcgatcaccgcttccctcatgatgtttaactttgttttagggcgactgccctgctgcgtaacatcgttgctgctccataacatcaaacatcgacccacggcgtaacgcgcttgctgcttggatgcccgaggcatagactgtaccccaaaaaaacagtcataacaagccatgaaaaccgccactgcgccgttaccaccgctgcgttcggtcaaggttctggaccagttgcgtgagcgcatacgctacttgcattacagcttacgaaccgaacaggcttatgtccactgggttcgtgccttcatccggatatcgacgtctgtgtggaattgtgagcggataacaaattcacacagggccctcggacaccgaggagaatgtcaagaggcgaacacacaacgtcttggagcgccagaggaggaacgagctaaaacggagcttttttgccctgcgtgaccagatcccggagttggaaaacaatgaaaatggctcgacagatccatttaaattttcaccgtcatcaccgaaacgcgcgaggcagctgtgcgtgaggctccggtgcccgtcagtgggcagagcgcacatcgcccacagtccccgagaagttggggggaggggtcggcaattgaaccggtgcctagagaaggtggcgcggggtaaactgggaaagtgatgtcgtgtactggctccgcctttttcccgagggtgggggagaaccgtatataagtgcagtagtcgccgtgaacgttctttttcgcaacgggtttgccgccagaacacaggtaagtgccgtgtgtggttcccgcgggcctggcctctttacgggttatggcccttgcgtgccttgaattacttccacctggctgcagtacgtgattcttgatcccgagcttcgggttggaagtgggtgggagagttcgaggccttgcgcttaaggagccccttcgcctcgtgcttgagttgaggcctggcctgggcgctggggccgccgcgtgcgaatctggtggcaccttcgcgcctgtctcgctgctttcgataagtctctagccatttaaaatttttgatgacctgctgcgacgctttttttctggcaagatagtcttgtaaatgcgggccaagatctgcacactggtatttcggtttttggggccgcgggcggcgacggggcccgtgcgtcccagcgcacatgttcggcgaggcggggcctgcgagcgcggccaccgagaatcggacgggggtagtctcaagctggccggcctgctctggtgcctggcctcgcgccgccgtgtatcgccccgccctgggcggcaaggctggcccggtcggcaccagttgcgtgagcggaaagatggccgcttcccggccctgctgcagggagctcaaaatggaggacgcggcgctcgggagagcgggcgggtgagtcacccacacaaaggaaaagggcctttccgtcctcagccgtcgcttcatgtgactccacggagtaccgggcgccgtccaggcacctcgattagttctcgagcttttggagtacgtcgtctttaggttggggggaggggttttatgcgatggagtttccccacactgagtgggtggagactgaagttaggccagcttggcacttgatgtaattctccttggaatttgccctttttgagtttggatcttggttcattctcaagcctcagacagtggttcaaagtttttttcttccatttcaggtgtcgtgaaattcgagctcggtacccccaaacttgacggcaatcctagcgtgaaggctggtaggattttatccccgctgccatcatggttcgaccattgaactgcatcgtcgccgtgtcccaaaatatggggattggcaagaacggagaccgaccctggcctccgctcaggaacgagttcaagtacttccaaagaatgaccacaacctcttcagtggaaggtaaacagaatctggtgattatgggtaggaaaacctggttctccattcctgagaagaatcgacctttaaaggacagaattaatatagttctcagtagagaactcaaagaaccaccacgaggagctcattttcttgccaaaagtttggatgatgccttaagacttattgaacaaccggaattggcaagtaaagtagacatggtttggatagtcggaggcagttctgtttaccaggaagccatgaatcaaccaggccacctcagactctttgtgacaaggatcatgcaggaatttgaaagtgacacgtttttcccagaaattgatttggggaaatataaacttctcccagaatacccaggcgtcctctctgaggtccaggaggaaaaaggcatcaagtataagtttgaagtctacgagaagaaagactaacaggaagatgctttcaagttctctgctcccctcctaaagctatgcatttttataagaccatgggggatgctcgatcccctcgcgagttggttcagctgctgcctgaggctggacgacctcgcggagttctaccggcagtgcaaatccgtcggcatccaggaaaccagcagcggctatccgcgcatccatgcccccgaactgcaggagtggggaggcacgatggccgctttggtccggatctttgtgaaggaaccttacttctgtggtgtgacataattggacaaactacctacagagatttaaagctctaaggtaaatataaaatttttaagtgtataatgtgttaaactactgattctaattgtttgtgtattttagattccaacctatggaactgatgaatgggagcagtggtggaatgcctttaatgaggaaaacctgttttgctcagaagaaatgccatctagtgatgatgaggctactgctgactctcaacattctactcctccaaaaaagaagagaaaggtagaagaccccaaggactttccttcagaattgctaagttttttgagtcatgctgtgtttagtaatagaactcttgcttgctttgctatttacaccacaaaggaaaaagctgcactgctatacaagaaaattatggaaaaatattctgtaacctttataagtaggcataacagttataatcataacatactgttttttcttactccacacaggcatagagtgtctgctattaataactatgctcaaaaattgtgtacctttagctttttaatttgtaaaggggttaataaggaatatttgatgtatagtgccttgactagaactcctcaggtgcaggctgcctatcagaaggtggtggctggtgtggccaatgccctggctcacaaataccactgagatctttttccctctgccaaaaattatggggacatcatgaagccccttgagcatctgacttctggctaataaaggaaatttattttcattgcaatagtgtgttggaattttttgtgtctctcactcggaaggacatatgggagggcaaatcatttaaaacatcagaatgagtatttggtttagagtttggcaacatatgcccatatgctggctgccatgaacaaaggttggctataaagaggtcatcagtatatgaaacagccccctgctgtccattccttattccatagaaaagccttgacttgaggttagattttttttatattttgttttgtgttatttttttctttaacatccctaaaattttccttacatgttttactagccagatttttcctcctctcctgactactcccagtcatagctgtccctcttctcttatggagatccctcgacg

SEQ ID NO: 7 - DNA, 9709 bp, Artificial Sequence
  synthetic vector sequence
aattcggatctggctccggtgcccgtcagtgggcagagcgcacatcgcccacagtccccgagaagttggggggaggggtcggcaattgaaccggtgcctagagaaggtggcgcggggtaaactgggaaagtgatgtcgtgtactggctccgcctttttcccgagggtgggggagaaccgtatataagtgcagtagtcgccgtgaacgttctttttcgcaacgggtttgccgccagaacacaggtaagtgccgtgtgtggttcccgcgggcctggcctctttacgggttatggcccttgcgtgccttgaattacttccacctggctgcagtacgtgattcttgatcccgagcttcgggttggaagtgggtgggagagttcgaggccttgcgcttaaggagccccttcgcctcgtgcttgagttgaggcctggcctgggcgctggggccgccgcgtgcgaatctggtggcaccttcgcgcctgtctcgctgctttcgataagtctctagccatttaaaatttttgatgacctgctgcgacgctttttttctggcaagatagtcttgtaaatgcgggccaagatctgcacactggtatttcggtttttggggccgcgggcggcgacggggcccgtgcgtcccagcgcacatgttcggcgaggcggggcctgcgagcgcggccaccgagaatcggacgggggtagtctcaagctggccggcctgctctggtgcctggtctcgcgccgccgtgtatcgccccgccctgggcggcaaggctggcccggtcggcaccagttgcgtgagcggaaagatggccgcttcccggccctgctgcagggagctcaaaatggaggacgcggcgctcgggagagcgggcgggtgagtcacccacacaaaggaaaagggcctttccgtcctcagccgtcgcttcatgtgactccacggagtaccgggcgccgtccaggcacctcgattagttctcgagcttttggagtacgtcgtctttaggttggggggaggggttttatgcgatggagtttccccacactgagtgggtggagactgaagttaggccagcttggcacttgatgtaattctccttggaatttgccctttttgagtttggatcttggttcattctcaagcctcagacagtggttcaaagtttttttcttccatttcaggtgtcgtgactcctgggcagtgtccactcccaggtccaactgcacctcggttctatcgaaaacgcgtccaccatgacccggctgaccgtgctggccctgctggccggcctgctggcctcctcccgggccctgcccgcccaggtggccttcaccccctacgcccccgagcccggctccacctgccggctgcgggagtactacgaccagaccgcccagatgtgctgctccaagtgctcccccggccagcacgccaaggtgttctgcaccaagacctccgacaccgtgtgcgactcctgcgaggactccacctacacccagctgtggaactgggtgcccgagtgcctgtcctgcggctcccggtgctcctccgaccaggtggagacccaggcctgcacccgggagcagaaccggatctgcacctgccggcccggctggtactgcgccctgtccaagcaggagggctgccggctgtgcgcccccctgcggaagtgccggcccggcttcggcgtggcccggcccggcaccgagacctccgacgtggtgtgcaagccctgcgcccccggcaccttctccaacaccacctcctccaccgacatctgccggccccaccagatctgcaacgtggtggccatccccggcaacgcctccatggacgccgtgtgcacctccacctcccccacccggtccatggcccccggcgccgtgcacctgccccagcccgtgtccacccggtcccagcacacccagcccacccccgagccctccaccgccccctccacctccttcctgctgcccatgggcccctccccccccgccgagggctccaccggcgacgagcccaagtcctgcgacaagacccacacctgccccccctgccccgcccccgagctgctgggcggcccctccgtgttcctgttcccccccaagcccaaggacaccctgatgatctcccggacccccgaggtgacctgcgtggtggtggacgtgtcccacgaggaccccgaggtgaagttcaactggtacgtggacggcgtggaggtgcacaacgccaagaccaagccccgggaggagcagtacaactccacctaccgggtggtgtccgtgctgaccgtgctgcaccaggactggctgaacggcaaggagtacaagtgcaaggtgtccaacaaggccctgcccgcccccatcgagaagaccatctccaaggccaagggccagccccgggagccccaggtgtacaccctgcccccctcccgggaggagatgaccaagaaccaggtgtccctgacctgcctggtgaagggcttctacccctccgacatcgccgtggagtgggagtccaacggccagcccgagaacaactacaagaccaccccccccgtgctggactccgacggctccttcttcctgtactccaagctgaccgtggacaagtcccggtggcagcagggcaacgtgttctcctgctccgtgatgcacgaggccctgcacaaccactacacccagaagtccctgtccctgtcccccggcaagtgatgaggcgcgccgggcggccgcttccctttagtgagggttaatgcttcgaggatgagtcgacccgggcggccgcttccctttagtgagggttaatgcttcgagactcctcaggtgcaggctgcctatcagaaggtggtggctggtgtggccaatgccctggctcacaaataccactgagatctttttccctctgccaaaaattatggggacatcatgaagccccttgagcatctgacttctggctaataaaggaaatttattttcattgcaatagtgtgttggaattttttgtgtctctcactcggaaggacatatgggagggcaaatcatttaaaacatcagaatgagtatttggtttagagtttggcaacatatgcccatatgctggctgccatgaacaaaggttggctataaagaggtcatcagtatatgaaacagccccctgctgtccattccttattccatagaaaagccttgacttgaggttagattttttttatattttgttttgtgttatttttttctttaacatccctaaaattttccttacatgttttactagccagatttttcctcctctcctgactactcccagtcatagctgtccctcttctcttatggagatccctcgacaaatccgataaggatcgatccgggctggcgtaatagcgaagaggcccgcaccgatcgcccttcccaacagttgcgcagcctgaatggcgaatggacgcgccctgtagcggcgcattaagcgcggcgggtgtggtggttacgcgcagcgtgaccgctacacttgccagcgccctagcgcccgctcctttcgctttcttcccttcctttctcgccacgttcgccggctttccccgtcaagctctaaatcgggggctccctttagggttccgatttagagctttacggcacctcgaccgcaaaaaacttgatttgggtgatggttcacgtagtgggccatcgccctgatagacggtttttcgccctttgacgttggagtccacgttctttaatagtggactcttgttccaaactggaacaacactcaaccctatctcggtctattcttttgatttataagggattttgccgatttcggcctattggttaaaaaatgagctgatttaacaaatatttaacgcgaattttaacaaaatattaacgtttacaatttcgcctgatgcggtattttctccttacgcatctgtgcggtatttcacaccgcatacgcggatctggtgtggaaagtccccaggctccccagcaggcagaagtatgcaaagcatgcatctcaattagtcagcaaccaggtgtggaaagtccccaggctccccagcaggcagaagtatgcaaagcatgcatctcaattagtcagcaaccatagtcccgcccctaactccgcccatcccgcccctaactccgcccagttccgcccattctccgccccatggctgactaattttttttatttatgcagaggccgaggccgcctcggcctctgagctattccagaagtagtgaggaggcttttttggaggcctaggcttttgcaaagatcgatcaagagacaggatgaggatcgtttcgcgctagcgctaccggtcgccaccatgattgaacaagatggattgcacgcaggttctccggccgcttgggtggagaggctattcggctatgactgggcacaacagacaatcggctgctctgatgccgccgtgttccggctgtcagcgcaggggcgcccggttctttttgtcaagaccgacctgtccggtgccctgaatgaactgcaggacgaggcagcgcggctatcgtggctggccacgacgggcgttccttgcgcagctgtgctcgacgttgtcactgaagcgggaagggactggctgctattgggcgaagtgccggggcaggatctcctgtcatctcaccttgctcctgccgagaaagtatccatcatggctgatgcaatgcggcggctgcatacgcttgatccggctacctgcccattcgaccaccaagcgaaacatcgcatcgagcgagcacgtactcggatggaagccggtcttgtcgatcaggatgatctggacgaagagcatcaggggctcgcgccagccgaactgttcgccaggctcaaggcgcgcatgcccgacggcgaggatctcgtcgtgacccatggcgatgcctgcttgccgaatatcatggtggaaaatggccgcttttctggattcatcgactgtggccggctgggtgtggcggaccgctatcaggacatagcgttggctacccgtgatattgctgaagagcttggcggcgaatgggctgaccgcttcctcgtgctttacggtatcgccgctcccgattcgcagcgcatcgccttctatcgccttcttgacgagttcttctgaaagcgggactctggggttcgaaatgaccgaccaagcgacgcccaacctgccatcacgagatttcgattccaccgccgccttctatgaaaggttgggcttcggaatcgttttccgggacgccggctggatgatcctccagcgcggggatctcatgctggagttcttcgcccaccccaacttgtttattgcagcttataatggttacaaataaagcaatagcatcacaaatttcacaaataaagcatttttttcactgcattctagttgtggtttgtccaaactcatcaatgtatcttatcatgtctgaatcgatagcgataaggatccgcgtatggtgcactctcggttgccgccgggcgttttttattggtgagaatcctcaggttactcatatatactttagattgatttaaaacttcatttttaatttaaaaggatctaggtgaagatcctttttgataatctcatgaccaaaatcccttaacgtgagttttcgttccactgagcgtcagaccccgtagaaaagatcaaaggatcttcttgagatcctttttttctgcgcgtaatctgctgcttgcaaacaaaaaaaccaccgctaccagcggtggtttgtttgccggatcaagagctaccaactctttttccgaaggtaactggcttcagcagagcgcagataccaaatactgtccttctagtgtagccgtagttaggccaccacttcaagaactctgtagcaccgcctacatacctcgctctgctaatcctgttaccagtggctgctgccagtggcgataagtcgtgtcttaccgggttggactcaagacgatagttaccggataaggcgcagcggtcgggctgaacggggggttcgtgcacacagcccagcttggagcgaacgacctacaccgaactgagatacctacagcgtgagctatgagaaagcgccacgcttcccgaagggagaaaggcggacaggtatccggtaagcggcagggtcggaacaggagagcgcacgagggagcttccagggggaaacgcctggtatctttatagtcctgtcgggtttcgccacctctgacttgagcgtcgatttttgtgatgctcgtcaggggggcggagcctatggaaaaacgccagcaacgcggcctttttacggttcctggccttttgctggccttttgctcacatgttctttcctgcgttatcccctgattctgtggataaccgtattaccgccatgcattagttattaagaccaataaaaaacgcccggcggcaaccgagcgttctgaacaaatccagatggagttctgaggtcattactggatctatcaacaggagtccaagcgagctcgatatcaaattacgccccgccctgccactcatcgcagtactgttgtaattcattaagcattctgccgacatggaagccatcacaaacggcatgatgaacctgaatcgccagcggcatcagcaccttgtcgccttgcgtataatatttgcccatggtgaaaacgggggcgaagaagttgtccatattggccacgtttaaatcaaaactggtgaaactcacccagggattggctgaaacgaaaaacatattctcaataaaccctttagggaaataggccaggttttcaccgtaacacgccacatcttgcgaatatatgtgtagaaactgccggaaatcgtcgtggtattcactccagagcgatgaaaacgtttcagtttgctcatggaaaacggtgtaacaagggtgaacactatcccatatcaccagctcaccgtctttcattgccatacgaaattccggatgagcattcatcaggcgggcaagaatgtgaataaaggccggataaaacttgtgcttatttttctttacggtctttaaaaaggccgtaatatccagctgaacggtctggttataggtacattgagcaactgactgaaatgcctcaaaatgttctttacgatgccattgggatatatcaacggtggtatatccagtgatttttttctccattttagcttccttagctcctgaaaatctcgataactcaaaaaatacgcccggtagtgatcttatttcattatggtgaaagttggaacctcttacgtgccgatcaacgtctcattttcgccaaaagttggcccagggcttcccggtatcaacagggacaccaggatttatttattctgcgaagtgatcttccgtcacaggtatttattcggatttaaattttcaccgtcatcaccgaaacgcgcgaggcagctgtgtagttattaatagtaatcaattacggggtcattagttcatagcccatatatggagttccgcgttacataacttacggtaaatggcccgcctggctgaccgcccaacgacccccgcccattgacgtcaataatgacgtatgttcccatagtaacgccaatagggactttccattgacgtcaatgggtggagtatttacggtaaactgcccacttggcagtacatcaagtgtatcatatgccaagtacgccccctattgacgtcaatgacggtaaatggcccgcctggcattatgcccagtacatgaccttatgggactttcctacttggcagtacatctacgtattagtcatcgctattaccatggtgatgcggttttggcagtacatcaatgggcgtggatagcggtttgactcacggggatttccaagtctccaccccattgacgtcaatgggagtttgttttggcaccaaaatcaacgggactttccaaaatgtcgtaacaactccgccccattgacgcaaatgggcggtaggcgtgtacggtgggaggtctatataagcagagctggtttagtgaaccgtcagatcaattcgagctcggtacccccaaacttgacggcaatcctagcgtgaaggctggtaggattttatccccgctgccatcatggttcgaccattgaactgcatcgtcgccgtgtcccaaaatatggggattggcaagaacggagaccgaccctggcctccgctcaggaacgagttcaagtacttccaaagaatgaccacaacctcttcagtggaaggtaaacagaatctggtgattatgggtaggaaaacctggttctccattcctgagaagaatcgacctttaaaggacagaattaatatagttctcagtagagaactcaaagaaccaccacgaggagctcattttcttgccaaaagtttggatgatgccttaagacttattgaacaaccggaattggcaagtaaagtagacatggtttggatagtcggaggcagttctgtttaccaggaagccatgaatcaaccaggccacctcagactctttgtgacaaggatcatgcaggaatttgaaagtgacacgtttttcccagaaattgatttggggaaatataaacttctcccagaatacccaggcgtcctctctgaggtccaggaggaaaaaggcatcaagtataagtttgaagtctacgagaagaaagactaacaggaagatgctttcaagttctctgctcccctcctaaagctatgcatttttataagaccatgggggatgctcgatcccctcgcgagttggttcagctgctgcctgaggctggacgacctcgcggagttctaccggcagtgcaaatccgtcggcatccaggaaaccagcagcggctatccgcgcatccatgcccccgaactgcaggagtggggaggcacgatggccgctttggtccggatctttgtgaaggaaccttacttctgtggtgtgacataattggacaaactacctacagagatttaaagctctaaggtaaatataaaatttttaagtgtataatgtgttaaactactgattctaattgtttgtgtattttagattccaacctatggaactgatgaatgggagcagtggtggaatgcctttaatgaggaaaacctgttttgctcagaagaaatgccatctagtgatgatgaggctactgctgactctcaacattctactcctccaaaaaagaagagaaaggtagaagaccccaaggactttccttcagaattgctaagttttttgagtcatgctgtgtttagtaatagaactcttgcttgctttgctatttacaccacaaaggaaaaagctgcactgctatacaagaaaattatggaaaaatattctgtaacctttataagtaggcataacagttataatcataacatactgttttttcttactccacacaggcatagagtgtctgctattaataactatgctcaaaaattgtgtacctttagctttttaatttgtaaaggggttaataaggaatatttgatgtatagtgccttgactagcgactgtgccttctagttgccagccatctgttgtttgcccctcccccgtgccttccttgaccctggaaggtgccactcccactgtcctttcctaataaaatgaggaaattgcatcgcattgtctgagtaggtgtcattctattctggggggtggggtggggcaggacagcaagggggaggattgggaagacaatagcaggcatgctggggatgcggtgggctctatggag

SEQ ID NO: 8 - DNA, 8967 bp, Artificial Sequence
  synthetic vector sequence
  CDC (1120)..(2526): "n" can mean any nucleotide, as long as the resulting amino acid sequence is identical to the Etanercept var1 sequence. For more detials see description of application.
  misc_feature (1120)..(2525): n is a, c, g, or t
tcaatattggccattagccatattattcattggttatatagcataaatcaatattggctattggccattgcatacgttgtatctatatcataatatgtacatttatattggctcatgtccaatatgaccgccatgttggcattgattattgactagttattaatagtaatcaattacggggtcattagttcatagcccatatatggagttccgcgttacataacttacggtaaatggcccgcctggctgaccgcccaacgacccccgcccattgacgtcaataatgacgtatgttcccatagtaacgccaatagggactttccattgacgtcaatgggtggagtatttacggtaaactgcccacttggcagtacatcaagtgtatcatatgccaagtacgccccctattgacgtcaatgacggtaaatggcccgcctggcattatgcccagtacatgaccttatgggactttcctacttggcagtacatctacgtattagtcatcgctattaccatggtgatgcggttttggcagtacatcaatgggcgtggatagcggtttgactcacggggatttccaagtctccaccccattgacgtcaatgggagtttgttttggcaccaaaatcaacgggactttccaaaatgtcgtaacaactccgccccattgacgcaaatgggcggtaggcgtgtacggtgggaggtctatataagcagagctcgtttagtgaaccgtcagatcgcctggagacgccatccacgctgttttgacctccatagaagacaccgggaccgatccagcctccgcggccgggaacggtgcattggaacgcggattccccgtgccaagagtgacgtaagtaccgcctatagagtctataggcccacccccttggcttcgttagaacgcggctacaattaatacataaccttatgtatcatacacatacgatttaggtgacactatagaataacatccactttgcctttctctccacaggtgtccactcccaggtccaactgcacctcggttctatcgaaaacgcgtccaccatggcccccgtggccgtgtgggctgccctggccgtgggcctggaactgtgggccgctgcccacgccnnnnnnnnnnnnnnnnnnnnnnnnnnnnnnnnnnnnnnnnnnnnnnnnnnnnnnnnnnnnnnnnnnnnnnnnnnnnnnnnnnnnnnnnnnnnnnnnnnnnnnnnnnnnnnnnnnnnnnnnnnnnnnnnnnnnnnnnnnnnnnnnnnnnnnnnnnnnnnnnnnnnnnnnnnnnnnnnnnnnnnnnnnnnnnnnnnnnnnnnnnnnnnnnnnnnnnnnnnnnnnnnnnnnnnnnnnnnnnnnnnnnnnnnnnnnnnnnnnnnnnnnnnnnnnnnnnnnnnnnnnnnnnnnnnnnnnnnnnnnnnnnnnnnnnnnnnnnnnnnnnnnnnnnnnnnnnnnnnnnnnnnnnnnnnnnnnnnnnnnnnnnnnnnnnnnnnnnnnnnnnnnnnnnnnnnnnnnnnnnnnnnnnnnnnnnnnnnnnnnnnnnnnnnnnnnnnnnnnnnnnnnnnnnnnnnnnnnnnnnnnnnnnnnnnnnnnnnnnnnnnnnnnnnnnnnnnnnnnnnnnnnnnnnnnnnnnnnnnnnnnnnnnnnnnnnnnnnnnnnnnnnnnnnnnnnnnnnnnnnnnnnnnnnnnnnnnnnnnnnnnnnnnnnnnnnnnnnnnnnnnnnnnnnnnnnnnnnnnnnnnnnnnnnnnnnnnnnnnnnnnnnnnnnnnnnnnnnnnnnnnnnnnnnnnnnnnnnnnnnnnnnnnnnnnnnnnnnnnnnnnnnnnnnnnnnnnnnnnnnnnnnnnnnnnnnnnnnnnnnnnnnnnnnnnnnnnnnnnnnnnnnnnnnnnnnnnnnnnnnnnnnnnnnnnnnnnnnnnnnnnnnnnnnnnnnnnnnnnnnnnnnnnnnnnnnnnnnnnnnnnnnnnnnnnnnnnnnnnnnnnnnnnnnnnnnnnnnnnnnnnnnnnnnnnnnnnnnnnnnnnnnnnnnnnnnnnnnnnnnnnnnnnnnnnnnnnnnnnnnnnnnnnnnnnnnnnnnnnnnnnnnnnnnnnnnnnnnnnnnnnnnnnnnnnnnnnnnnnnnnnnnnnnnnnnnnnnnnnnnnnnnnnnnnnnnnnnnnnnnnnnnnnnnnnnnnnnnnnnnnnnnnnnnnnnnnnnnnnnnnnnnnnnnnnnnnnnnnnnnnnnnnnnnnnnnnnnnnnnnnnnnnnnnnnnnnnnnnnnnnnnnnnnnnnnnnnnnnnnnnnnnnnnnnnnnnnnnnnnnnnnnnnnnnnnnnnnnnnnnnnnnnnnnnnnnnnnnnnnnnnnnnnnnnnnnnnnnnnnnnnnnnnnnnnnnnnnnnnnnnnnnnnnnnnnnnnnnnnnnnnnnnnnnnnnnnnnnnnnnnnnnnnnnnnnnnnnnnnnnnnnnnnnnnnnnnnnnnnnnnnnnnnnnnnnnnnnnnnnnnnnnnnnnnnnnnnnnnnnnnnnnnnnnnnnnnnnnnnnnnnnnnnaggcgcgccgggcggccgcttccctttagtgagggttaatgcttcgagcagacatgataagatacattgatgagtttggacaaaccacaactagaatgcagtgaaaaaaatgctttatttgtgaaatttgtgatgctattgctttatttgtaaccattataagctgcaataaacaagttaacaacaacaattgcattcattttatgtttcaggttcagggggagatgtgggaggttttttaaagcaagtaaaacctctacaaatgtggtaaaatccgataaggatcgatccgggctggcgtaatagcgaagaggcccgcaccgatcgcccttcccaacagttgcgcagcctgaatggcgaatggacgcgccctgtagcggcgcattaagcgcggcgggtgtggtggttacgcgcagcgtgaccgctacacttgccagcgccctagcgcccgctcctttcgctttcttcccttcctttctcgccacgttcgccggctttccccgtcaagctctaaatcgggggctccctttagggttccgatttagagctttacggcacctcgaccgcaaaaaacttgatttgggtgatggttcacgtagtgggccatcgccctgatagacggtttttcgccctttgacgttggagtccacgttctttaatagtggactcttgttccaaactggaacaacactcaaccctatctcggtctattcttttgatttataagggattttgccgatttcggcctattggttaaaaaatgagctgatttaacaaatatttaacgcgaattttaacaaaatattaacgtttacaatttcgcctgatgcggtattttctccttacgcatctgtgcggtatttcacaccgcatacgcggatctgcgcagcaccatggcctgaaataacctctgaaagaggaacttggttaggtaccttctgaggcggaaagaaccagctgtggaatgtgtgtcagttagggtgtggaaagtccccaggctccccagcaggcagaagtatgcaaagcatgcatctcaattagtcagcaaccaggtgtggaaagtccccaggctccccagcaggcagaagtatgcaaagcatgcatctcaattagtcagcaaccatagtcccgcccctaactccgcccatcccgcccctaactccgcccagttccgcccattctccgccccatggctgactaattttttttatttatgcagaggccgaggccgcctcggcctctgagctattccagaagtagtgaggaggcttttttggaggcctaggcttttgcaaaaagcttgattcttctgacacaacagtctcgaacttaaggctagagccaccatgattgaacaagatggattgcacgcaggttctccggccgcttgggtggagaggctattcggctatgactgggcacaacagacaatcggctgctctgatgccgccgtgttccggctgtcagcgcaggggcgcccggttctttttgtcaagaccgacctgtccggtgccctgaatgaactgcaggacgaggcagcgcggctatcgtggctggccacgacgggcgttccttgcgcagctgtgctcgacgttgtcactgaagcgggaagggactggctgctattgggcgaagtgccggggcaggatctcctgtcatctcaccttgctcctgccgagaaagtatccatcatggctgatgcaatgcggcggctgcatacgcttgatccggctacctgcccattcgaccaccaagcgaaacatcgcatcgagcgagcacgtactcggatggaagccggtcttgtcgatcaggatgatctggacgaagagcatcaggggctcgcgccagccgaactgttcgccaggctcaaggcgcgcatgcccgacggcgaggatctcgtcgtgacccatggcgatgcctgcttgccgaatatcatggtggaaaatggccgcttttctggattcatcgactgtggccggctgggtgtggcggaccgctatcaggacatagcgttggctacccgtgatattgctgaagagcttggcggcgaatgggctgaccgcttcctcgtgctttacggtatcgccgctcccgattcgcagcgcatcgccttctatcgccttcttgacgagttcttctgagcgggactctggggttcgaaatgaccgaccaagcgacgcccaacctgccatcacgatggccgcaataaaatatctttattttcattacatctgtgtgttggttttttgtgtgaatcgatagcgataaggatccgcgtatggtgcactctcagtacaatctgctctgatgccgcatagttaagccagccccgacacccgccaacacccgctgacgcgccctgacgggcttgtctgctcccggcatccgcttacagacaagctgtgaccgtctccgggagctgcatgtgtcagaggttttcaccgtcatcaccgaaacgcgcgagacgaaagggcctcgtgatacgcctatttttataggttaatgtcatgataataatggtttcttagacgtcaggtggcacttttcggggaaatgtgcgcggaacccctatttgtttatttttctaaatacattcaaatatgtatccgctcatgagacaataaccctgataaatgcttcaataatattgaaaaaggaagagtatgagtattcaacatttccgtgtcgcccttattcccttttttgcggcattttgccttcctgtttttgctcacccagaaacgctggtgaaagtaaaagatgctgaagatcagttgggtgcacgagtgggttacatcgaactggatctcaacagcggtaagatccttgagagttttcgccccgaagaacgttttccaatgatgagcacttttaaagttctgctatgtggcgcggtattatcccgtattgacgccgggcaagagcaactcggtcgccgcatacactattctcagaatgacttggttgagtactcaccagtcacagaaaagcatcttacggatggcatgacagtaagagaattatgcagtgctgccataaccatgagtgataacactgcggccaacttacttctgacaacgatcggaggaccgaaggagctaaccgcttttttgcacaacatgggggatcatgtaactcgccttgatcgttgggaaccggagctgaatgaagccataccaaacgacgagcgtgacaccacgatgcctgtagcaatggcaacaacgttgcgcaaactattaactggcgaactacttactctagcttcccggcaacaattaatagactggatggaggcggataaagttgcaggaccacttctgcgctcggcccttccggctggctggtttattgctgataaatctggagccggtgagcgtgggtctcgcggtatcattgcagcactggggccagatggtaagccctcccgtatcgtagttatctacacgacggggagtcaggcaactatggatgaacgaaatagacagatcgctgagataggtgcctcactgattaagcattggtaactgtcagaccaagtttactcatatatactttagattgatttaaaacttcatttttaatttaaaaggatctaggtgaagatcctttttgataatctcatgaccaaaatcccttaacgtgagttttcgttccactgagcgtcagaccccgtagaaaagatcaaaggatcttcttgagatcctttttttctgcgcgtaatctgctgcttgcaaacaaaaaaaccaccgctaccagcggtggtttgtttgccggatcaagagctaccaactctttttccgaaggtaactggcttcagcagagcgcagataccaaatactgtccttctagtgtagccgtagttaggccaccacttcaagaactctgtagcaccgcctacatacctcgctctgctaatcctgttaccagtggctgctgccagtggcgataagtcgtgtcttaccgggttggactcaagacgatagttaccggataaggcgcagcggtcgggctgaacggggggttcgtgcacacagcccagcttggagcgaacgacctacaccgaactgagatacctacagcgtgagctatgagaaagcgccacgcttcccgaagggagaaaggcggacaggtatccggtaagcggcagggtcggaacaggagagcgcacgagggagcttccagggggaaacgcctggtatctttatagtcctgtcgggtttcgccacctctgacttgagcgtcgatttttgtgatgctcgtcaggggggcggagcctatggaaaaacgccagcaacgcggcctttttacggttcctggccttttgctggccttttgctcacatggctcgacagatccatttaaattttcaccgtcatcaccgaaacgcgcgaggcagctgtggaatgtgtgtcagttagggtgtggaaagtccccaggctccccagcaggcagaagtatgcaaagcatgcatctcaattagtcagcaaccaggtgtggaaagtccccaggctccccagcaggcagaagtatgcaaagcatgcatctcaattagtcagcaaccatagtcccgcccctaactccgcccatcccgcccctaactccgcccagttccgcccattctccgccccatggctgactaattttttttatttatgcagaggccgaggccgcctcggcctctgagctattccagaagtagtgaggaggcttttttggaggcctaggcttttgcaaaaagctaattcgagctcggtacccccaaacttgacggcaatcctagcgtgaaggctggtaggattttatccccgctgccatcatggttcgaccattgaactgcatcgtcgccgtgtcccaaaatatggggattggcaagaacggagaccgaccctggcctccgctcaggaacgagttcaagtacttccaaagaatgaccacaacctcttcagtggaaggtaaacagaatctggtgattatgggtaggaaaacctggttctccattcctgagaagaatcgacctttaaaggacagaattaatatagttctcagtagagaactcaaagaaccaccacgaggagctcattttcttgccaaaagtttggatgatgccttaagacttattgaacaaccggaattggcaagtaaagtagacatggtttggatagtcggaggcagttctgtttaccaggaagccatgaatcaaccaggccacctcagactctttgtgacaaggatcatgcaggaatttgaaagtgacacgtttttcccagaaattgatttggggaaatataaacttctcccagaatacccaggcgtcctctctgaggtccaggaggaaaaaggcatcaagtataagtttgaagtctacgagaagaaagactaacaggaagatgctttcaagttctctgctcccctcctaaagctatgcatttttataagaccatgggggatgctcgatcccctcgcgagttggttcagctgctgcctgaggctggacgacctcgcggagttctaccggcagtgcaaatccgtcggcatccaggaaaccagcagcggctatccgcgcatccatgcccccgaactgcaggagtggggaggcacgatggccgctttggtccgagatctttgtgaaggaaccttacttctgtggtgtgacataattggacaaactacctacagagatttaaagctctaaggtaaatataaaatttttaagtgtataatgtgttaaactactgattctaattgtttgtgtattttagattccaacctatggaactgatgaatgggagcagtggtggaatgcctttaatgaggaaaacctgttttgctcagaagaaatgccatctagtgatgatgaggctactgctgactctcaacattctactcctccaaaaaagaagagaaaggtagaagaccccaaggactttccttcagaattgctaagttttttgagtcatgctgtgtttagtaatagaactcttgcttgctttgctatttacaccacaaaggaaaaagctgcactgctatacaagaaaattatggaaaaatattctgtaacctttataagtaggcataacagttataatcataacatactgttttttcttactccacacaggcatagagtgtctgctattaataactatgctcaaaaattgtgtacctttagctttttaatttgtaaaggggttaataaggaatatttgatgtatagtgccttgactagagatcataatcagccataccacatttgtagaggttttacttgctttaaaaaacctcccacacctccccctgaacctgaaacataaaatgaatgcaattgttgttgttaacttgtttattgcagcttataatggttacaaataaagcaatagcatcacaaatttcacaaataaagcattttttcactgcattctagttgtggtttgaattcggatct

SEQ ID NO: 9 - protein, 10 aa, arteficail sequence
RSLLSLRSSL

SEQ ID NO: 10 - protein, 10 aa, wikipedia genetic code
MHVAWNDMCP